European Patent Application EP 4 442 830 A1, published October 9, 2024. Title: AADC/GDNF POLYNUCLEOTIDE, AND USE THEREOF IN TREATING PARKINSON'S DISEASE. Applicant: Shanghai Regenelead Therapies Co.,LTD. Application CN PCT/CN2022/134993, filed November 29, 2022. The sequence listing filed with the application follows.

SEQUENCE LISTING (50 sequences)

SEQ ID NO: 1 - protein, 480 aa, synthetic construct
  source 1..480: note = AADC
MNASEFRRRGKEMVDYVANYMEGIEGRQVYPDVEPGYLRPLIPAAAPQEPDTFEDIINDVEKIIMPGVTHWHSPYFFAYFPTASSYPAMLADMLCGAIGCIGFSWAASPACTELETVMMDWLGKMLELPKAFLNEKAGEGGGVIQGSASEATLVALLAARTKVIHRLQAASPELTQAAIMEKLVAYSSDQAHSSVERAGLIGGVKLKAIPSDGNFAMRASALQEALERDKAAGLIPFFMVATLGTTTCCSFDNLLEVGPICNKEDIWLHVDAAYAGSAFICPEFRHLLNGVEFADSFNFNPHKWLLVNFDCSAMWVKKRTDLTGAFRLDPTYLKHSHQDSGLITDYRHWQIPLGRRFRSLKMWFVFRMYGVKGLQAYIRKHVQLSHEFESLVRQDPRFEICVEVILGLVCFRLKGSNKVNEALLQRINSAKKIHLVPCHLRDKFVLRFAICSRTVESAHVQRAWEHIKELAADVLRAERE

SEQ ID NO: 2 - protein, 211 aa, synthetic construct
  source 1..211: note = GDNF
MKLWDVVAVCLVLLHTASAFPLPAGKRPPEAPAEDRSLGRRRAPFALSSDSNMPEDYPDQFDDVMDFIQATIKRLKRSPDKQMAVLPRRERNRQAAAANPENSRGKGRRGQRGKNRGCVLTAIHLNVTDLGLGYETKEELIFRYCSGSCDAAETTYDKILKNLSRNRRLVSDKVGQACCRPIAFDDDLSFLDDNLVYHILRKHSAKRCGCI

SEQ ID NO: 3 - DNA, 1443 bp, Homo sapiens
  source 1..1443: mol_type = genomic DNA; note = AADC(WT)
atgaacgcaagtgaattccgaaggagagggaaggagatggtggattacatggccaactacatggaaggcattgagggacgccaggtctaccctgacgtggagcccgggtacctgcggccgctgatccctgccgctgcccctcaggagccagacacgtttgaggacatcatcaacgacgttgagaagataatcatgcctggggtgacgcactggcacagcccctacttcttcgcctacttccccactgccagctcgtacccggccatgcttgcggacatgctgtgcggggccattggctgcatcggcttctcctgggcggcaagcccagcatgcacagagctggagactgtgatgatggactggctcgggaagatgctggaactaccaaaggcatttttgaatgagaaagctggagaagggggaggagtgatccagggaagtgccagtgaagccaccctggtggccctgctggccgctcggaccaaagtgatccatcggctgcaggcagcgtccccagagctcacacaggccgctatcatggagaagctggtggcttactcatccgatcaggcacactcctcagtggaaagagctgggttaattggtggagtgaaattaaaagccatcccctcagatggcaacttcgccatgcgtgcgtctgccctgcaggaagccctggagagagacaaagcggctggcctgattcctttctttatggttgccaccctggggaccacaacatgctgctcctttgacaatctcttagaagtcggtcctatctgcaacaaggaagacatatggctgcacgttgatgcagcctacgcaggcagtgcattcatctgccctgagttccggcaccttctgaatggagtggagtttgcagattcattcaactttaatccccacaaatggctattggtgaattttgactgttctgccatgtgggtgaaaaagagaacagacttaacgggagcctttagactggaccccacttacctgaagcacagccatcaggattcagggcttatcactgactaccggcattggcagataccactgggcagaagatttcgctctttgaaaatgtggtttgtatttaggatgtatggagtcaaaggactgcaggcttatatccgcaagcatgtccagctgtcccatgagtttgagtcactggtgcgccaggatccccgctttgaaatctgtgtggaagtcattctggggcttgtctgctttcggctaaagggttccaacaaagtgaatgaagctcttctgcaaagaataaacagtgccaaaaaaatccacttggttccatgtcacctcagggacaagtttgtcctgcgctttgccatctgttctcgcacggtggaatctgcccatgtgcagcgggcctgggaacacatcaaagagctggcggccgacgtgctgcgagcagagagggagtag

SEQ ID NO: 4 - DNA, 1443 bp, synthetic construct
  source 1..1443: mol_type = other DNA; note = AADC01
atgaatgctagcgagtttcgcagaaggggcaaggagatggtggattacgtggctaattacatggagggcatcgagggccggcaggtgtacccagatgtggagccaggctacctgagaccactgatccctgctgccgccccacaggagccagacaccttcgaggatatcatcaatgacgtggagaagatcatcatgcctggcgtgacccactggcatagcccatacttctttgcctactttccaacagcctcttcctatcccgctatgctggctgatatgctgtgcggcgctatcggctgcatcggcttctcttgggccgctagccctgcttgcacagagctggagaccgtgatgatggattggctgggcaagatgctggagctgcctaaggcctttctgaacgagaaggctggcgagggcggcggcgtgatccagggctctgcctccgaggctacactggtggctctgctggctgcccggacaaaggtaatccacagactgcaggctgcctctccagagctgacccaggccgctatcatggagaagctggtggcttactctagcgaccaggctcattcttccgtggagcgggctggcctgatcggcggcgtgaagctgaaggccatcccttccgacggcaatttcgccatgagagcttctgccctgcaggaggctctggagagagataaggctgccggcctgatccctttctttatggtggccaccctgggcacaaccacctgttgctccttcgacaacctgctggaggtgggccctatctgtaacaaggaggacatctggctgcatgtggatgccgcttatgctggctctgcctttatctgccccgagtttagacatctgctgaacggcgtggagtttgccgacagctttaacttcaaccctcacaagtggctgctggtgaattttgactgctctgccatgtgggtgaagaagaggacagacctgaccggcgcttttaggctggatccaacctacctgaagcacagccatcaggacagcggcctgatcacagactacagacactggcagatcccactgggcagaaggtttcggtctctgaagatgtggttcgtgtttcgcatgtatggcgtgaagggcctgcaggcttatatccggaagcacgtgcagctgtctcatgagttcgagtccctggtgcggcaggacccaagatttgagatctgcgtggaggtaatcctgggcctggtgtgcttcaggctgaagggctctaataaggtgaacgaggctctgctgcagaggatcaacagcgccaagaagatccatctggtgccttgtcatctgagggacaagttcgtgctgagattcgccatctgctctagaacagtggagtctgctcatgtgcagagggcttgggagcatatcaaggagctggccgctgacgtgctgagggctgagagggagtga

SEQ ID NO: 5 - DNA, 1443 bp, synthetic construct
  source 1..1443: mol_type = other DNA; note = AADC02
atgaacgctagcgagtttcggaggagaggcaaggagatggtggactacgtggccaactacatggagggcatcgagggcagacaggtgtacccagacgtggagcctggctatctgcggccactgatccctgctgccgccccacaggagccagatacctttgaggacatcatcaacgacgtggagaagatcatcatgcccggcgtgacccactggcattccccttacttctttgcctactttcctacagcttcttcctatcctgccatgctggccgatatgctgtgcggcgctatcggctgcatcggcttctcttgggccgcttcccccgcttgcaccgagctggagaccgtgatgatggattggctgggcaagatgctggagctgcccaaggctttcctgaatgagaaggctggcgagggcggcggcgtgatccagggctctgcttccgaggccacactggtggccctgctggctgccaggacaaaggtaatccacagactgcaggctgcctcccccgagctgacccaggccgctatcatggagaagctggtggcttactcctctgaccaggctcactcttccgtggagagagctggcctgatcggcggcgtgaagctgaaggctatcccttctgatggcaatttcgccatgagggcttctgctctgcaggaggctctggagagggataaggctgccggcctgatcccctttttcatggtggccaccctgggcacaaccacctgttgcagctttgacaatctgctggaggtgggccctatctgcaacaaggaggacatctggctgcacgtggatgctgcctacgctggcagcgccttcatctgtcccgagtttaggcacctgctgaatggcgtggagtttgctgactcctttaatttcaacccccataagtggctgctggtgaacttcgactgctctgctatgtgggtgaagaagaggacagatctgacaggcgcctttaggctggacccaacctacctgaagcactcccatcaggatagcggcctgatcaccgactaccggcactggcagatccctctgggcaggcgctttagatccctgaagatgtggttcgtgtttaggatgtacggcgtgaagggcctgcaggcttatatccggaagcatgtgcagctgtcccacgagttcgagtctctggtgcggcaggacccaaggtttgagatctgcgtggaggtaatcctgggcctggtgtgcttcagactgaagggctccaataaggtgaacgaggctctgctgcagagaatcaactccgccaagaagatccacctggtgccttgtcacctgagggataagttcgtgctgaggtttgccatctgctctagaaccgtggagagcgcccatgtgcagagggcttgggagcacatcaaggagctggctgccgacgtgctgagggctgagagagagtga

SEQ ID NO: 6 - DNA, 1443 bp, synthetic construct
  source 1..1443: mol_type = other DNA; note = AADC03
atgaatgcctctgagttccgcagacgcggcaaggagatggtggactacgtggctaactacatggagggcatcgagggcagacaggtgtaccccgacgtggagcctggctatctgaggccactgatccctgctgctgcccctcaggagcccgacaccttcgaggatatcatcaatgacgtggagaagatcatcatgccaggcgtgacccattggcactctccatacttctttgcttacttccctaccgcctcttcctatccagctatgctggccgatatgctgtgcggcgccatcggctgcatcggctttagctgggctgcctctccagcttgtaccgagctggagacagtgatgatggactggctgggcaagatgctggagctgcctaaggcctttctgaacgagaaggccggcgagggcggcggcgtgatccagggctccgcttctgaggccaccctggtggctctgctggctgccagaaccaaggtaatccacaggctgcaggccgctagccctgagctgacccaggccgctatcatggagaagctggtggcttactcttccgaccaggcccattctagcgtggagagggctggcctgatcggcggcgtgaagctgaaggctatcccttctgacggcaacttcgccatgagagctagcgccctgcaggaggccctggagcgggacaaggctgccggcctgatcccatttttcatggtggctaccctgggcacaacaacctgctgttctttcgacaacctgctggaggtgggccctatctgcaataaggaggacatctggctgcatgtggatgctgcctatgctggcagcgcctttatctgcccagagttcaggcatctgctgaacggcgtggagtttgccgactcttttaacttcaatccccataagtggctgctggtgaactttgactgtagcgccatgtgggtgaagaagaggacagatctgaccggcgcctttcggctggatcctacctacctgaagcactctcatcaggattctggcctgatcaccgattacagacattggcagatccctctgggccggagatttcggagcctgaagatgtggttcgtgtttcggatgtatggcgtgaagggcctgcaggcctatatcagaaagcacgtgcagctgtcccacgagtttgagagcctggtgcgccaggacccacggtttgagatctgcgtggaggtaatcctgggcctggtgtgcttcaggctgaagggctctaataaggtgaacgaggctctgctgcagcgcatcaactccgctaagaagatccacctggtgccttgtcacctgcgggacaagttcgtgctgaggtttgccatctgctccagaaccgtggagtctgcccatgtgcagagagcttgggagcatatcaaggagctggccgctgatgtgctgagggctgagagagagtga

SEQ ID NO: 7 - DNA, 1443 bp, synthetic construct
  source 1..1443: mol_type = other DNA; note = AADC04
atgaacgcctctgagtttcggaggaggggcaaggagatggtggactacgtggctaactatatggagggcatcgagggcagacaggtgtaccctgacgtggagccaggctacctgagaccactgatcccagccgccgctcctcaggagcctgacacctttgaggacatcatcaatgatgtggagaagatcatcatgcctggcgtgacccattggcacagcccttactttttcgcctatttcccaaccgctagctcctatccagccatgctggctgatatgctgtgcggcgctatcggctgtatcggctttagctgggctgcctctcctgcttgtacagagctggagacagtgatgatggattggctgggcaagatgctggagctgcccaaggcctttctgaacgagaaggccggcgagggcggcggcgtgatccagggctctgcttctgaggccacactggtggctctgctggccgctaggaccaaggtaatccacaggctgcaggctgccagcccagagctgacccaggctgccatcatggagaagctggtggcctactctagcgaccaggctcattcctctgtggagagggctggcctgatcggcggcgtgaagctgaaggctatcccttccgatggcaatttcgctatgagagccagcgccctgcaggaggctctggagagggacaaggctgccggcctgatccctttcttcatggtggccacactgggcacaaccacatgctgttctttcgacaacctgctggaggtgggccccatctgcaataaggaggacatctggctgcatgtggatgctgcctacgccggctccgcttttatctgccctgagtttcggcatctgctgaacggcgtggagtttgccgacagctttaacttcaatccccacaagtggctgctggtgaacttcgactgctctgctatgtgggtgaagaagaggacagatctgaccggcgctttcagactggatccaacctacctgaagcactctcatcaggactctggcctgatcaccgattaccggcattggcagatccctctgggccgccggtttaggagcctgaagatgtggttcgtgtttcggatgtatggcgtgaagggcctgcaggcctatatccggaagcatgtgcagctgtctcatgagtttgagtccctggtgcgccaggaccctaggttcgagatctgcgtggaggtaatcctgggcctggtgtgcttcaggctgaagggcagcaataaggtgaacgaggctctgctgcagaggatcaattccgctaagaagatccacctggtgccttgtcatctgcgggataagtttgtgctgaggttcgccatctgtagccgcaccgtggagtctgcccacgtgcagagagcttgggagcacatcaaggagctggccgctgatgtgctgagagctgagagggagtga

SEQ ID NO: 8 - DNA, 636 bp, Homo sapiens
  source 1..636: mol_type = genomic DNA; note = GDNF(WT)
atgaagttatgggatgtcgtggctgtctgcctggtgctgctccacaccgcgtccgccttcccgctgcccgccggtaagaggcctcccgaggcgcccgccgaagaccgctccctcggccgccgccgcgcgcccttcgcgctgagcagtgactcaaatatgccagaggattatcctgatcagttcgatgatgtcatggattttattcaagccaccattaaaagactgaaaaggtcaccagataaacaaatggcagtgcttcctagaagagagcggaatcggcaggctgcagctgccaacccagagaattccagaggaaaaggtcggagaggccagaggggcaaaaaccggggttgtgtcttaactgcaatacatttaaatgtcactgacttgggtctgggctatgaaaccaaggaggaactgatttttaggtactgcagcggctcttgcgatgcagctgagacaacgtacgacaaaatattgaaaaacttatccagaaatagaaggctggtgagtgacaaagtagggcaggcatgttgcagacccatcgcctttgatgatgacctgtcgtttttagatgataacctggtttaccatattctaagaaagcattccgctaaaaggtgtggatgtatctga

SEQ ID NO: 9 - DNA, 636 bp, synthetic construct
  source 1..636: mol_type = other DNA; note = GDNF01
atgaagctgtgggatgtggtggccgtgtgcctggtgctgctgcatacagctagcgcctttcccctgccagctggcaagagaccacctgaggctcctgccgaggacagatctctgggcaggagacgggcccctttcgctctgtctagcgattccaacatgcccgaggactatccagaccagttcgatgacgtgatggacttcatccaggctaccatcaagaggctgaagagaagcccagacaagcagatggctgtgctgcctagacgcgagaggaatagacaggccgctgctgccaatcctgagaacagcaggggcaagggccggaggggccagcgcggcaagaatagaggctgcgtgctgaccgctatccacctgaacgtgacagacctgggcctgggctacgagaccaaggaggagctgatcttccgctattgttccggctcttgtgatgccgctgagaccacatatgacaagatcctgaagaacctgagcagaaacaggagactggtgtctgacaaggtgggccaggcctgttgcagaccaatcgccttcgatgatgacctgagctttctggacgataacctggtgtatcacatcctgagaaagcactctgccaagagatgtggctgcatctga

SEQ ID NO: 10 - DNA, 636 bp, synthetic construct
  source 1..636: mol_type = other DNA; note = GDNF02
atgaagctgtgggatgtggtggccgtgtgcctggtgctgctgcatacagcttctgcctttcctctgcccgctggcaagaggcctccagaggccccagctgaggacagatccctgggcagaaggagagccccttttgctctgtccagcgactctaacatgcccgaggattatcccgaccagttcgacgatgtgatggacttcatccaggctaccatcaagaggctgaagagaagcccagataagcagatggctgtgctgccacgcagagagaggaacagacaggccgctgctgctaaccctgagaactctcggggcaagggcagaaggggccagagaggcaagaatcgcggctgcgtgctgacagctatccacctgaacgtgacagatctgggcctgggctacgagacaaaggaggagctgatcttcagatactgttctggcagctgtgatgctgccgagacaacctacgacaagatcctgaagaacctgagcagaaatcggaggctggtgtccgataaggtgggccaggcctgttgcagacctatcgctttcgacgacgatctgagcttcctggacgataacctggtgtaccacatcctgcggaagcattctgccaagagatgcggctgtatctga

SEQ ID NO: 11 - DNA, 636 bp, synthetic construct
  source 1..636: mol_type = other DNA; note = GDNF03
atgaagctgtgggatgtggtggccgtgtgcctggtgctgctgcatacagcttctgccttccctctgccagctggcaagagaccacctgaggcccccgctgaggatagaagcctgggccgcagaagggctccttttgccctgagctccgactctaatatgcctgaggattacccagaccagttcgatgacgtgatggactttatccaggccacaatcaagcgcctgaagaggtctccagacaagcagatggctgtgctgcctaggagagagagaaaccggcaggctgccgctgctaatccagagaactctaggggcaagggcaggagaggccagaggggcaagaatcgcggctgcgtgctgaccgctatccatctgaatgtgaccgatctgggcctgggctacgagacaaaggaggagctgatcttcaggtactgcagcggctcttgtgacgccgctgagaccacatacgacaagatcctgaagaacctgagcagaaaccgcagactggtgtctgataaggtgggccaggcttgttgcaggcccatcgcttttgatgacgatctgtctttcctggacgataatctggtgtaccacatcctgcggaagcactctgctaagcggtgtggctgcatctga

SEQ ID NO: 12 - DNA, 636 bp, synthetic construct
  source 1..636: mol_type = other DNA; note = GDNF04
atgaagctgtgggatgtggtggccgtgtgcctggtgctgctgcacaccgcttctgccttcccactgcctgccggcaagagacctcccgaggcccctgccgaggacagaagcctgggcaggcggagagccccatttgctctgtctagcgattccaacatgcctgaggattaccccgatcagttcgatgacgtgatggatttcatccaggccaccatcaagagactgaagagatctcctgacaagcagatggctgtgctgcctagaagggagagaaacaggcaggccgctgctgccaatccagagaactccaggggcaagggcagaaggggccagcgcggcaagaatagaggctgcgtgctgacagccatccacctgaacgtgaccgacctgggcctgggctacgagaccaaggaggagctgatcttcaggtactgtagcggctcctgtgatgctgccgagaccacatacgacaagatcctgaagaacctgtccaggaacagaaggctggtgtctgacaaggtgggccaggcttgctgtaggccaatcgctttcgacgacgatctgtcctttctggatgacaacctggtgtaccacatcctgaggaagcattccgctaagagatgtggctgcatctga

SEQ ID NO: 13 - DNA, 3064 bp, synthetic construct
  source 1..3064: mol_type = other DNA; note = HRPDAAV01-A
cctgcaggcagctgcgcgctcgctcgctcactgaggccgcccgggcaaagcccgggcgtcgggcgacctttggtcgcccggcctcagtgagcgagcgagcgcgcagagagggagtggccaactccatcactaggggttcctatcgatatcaagcttcgttacataacttacggtaaatggcccgcctggctgaccgcccaacgacccccgcccattgacgtcaatagtaacgccaatagggactttccattgacgtcaatgggtggagtatttacggtaaactgcccacttggcagtacatcaagtgtatcatatgccaagtacgccccctattgacgtcaatgacggtaaatggcccgcctggcattgtgcccagtacatgaccttatgggactttcctacttggcagtacatctacgtattagtcatcgctattaccatggtcgaggtgagccccacgttctgcttcactctccccatctcccccccctccccacccccaattttgtatttatttattttttaattattttgtgcagcgatgggggcggggggggggggggggcgcgcgccaggcggggcggggcggggcgaggggcggggcggggcgaggcggagaggtgcggcggcagccaatcagagcggcgcgctccgaaagtttccttttatggcgaggcggcggcggcggcggccctataaaaagcgaagcgcgcggcgggcgggagtcgctgcgcgctgccttcgccccgtgccccgctccgccgccgcctcgcgccgcccgccccggctctgactgaccgcgttactcccacaggtgagcgggcgggacggcccttctcctccgggctgtaattagctgagcaagaggtaagggtttaagggatggttggttggtggggtattaatgtttaattacctggagcacctgcctgaaatcactttttttcaggttgggggattcgaacatcggccgccaccatgaacgccagcgagttcaggaggaggggcaaggagatggtggactacgtggccaactacatggagggcatcgagggcaggcaggtgtaccccgacgtggagcccggctacctgaggcccctgatccccgccgccgccccccaggagcccgacaccttcgaggacatcatcaacgacgtggagaagatcatcatgcccggcgtgacccactggcacagcccctacttcttcgcctacttccccaccgccagcagctaccccgccatgctggccgacatgctgtgcggcgccatcggctgcatcggcttcagctgggccgccagccccgcctgcaccgagctggagaccgtgatgatggactggctgggcaagatgctggagctgcccaaggccttcctgaacgagaaggccggcgagggcggcggcgtgatccagggcagcgccagcgaggccaccctggtggccctgctggccgccaggaccaaggtgatccacaggctgcaggccgccagccccgagctgacccaggccgccatcatggagaagctggtggcctacagcagcgaccaggcccacagcagcgtggagagggccggcctgatcggcggcgtgaagctgaaggccatccccagcgacggcaacttcgccatgagggccagcgccctgcaggaggccctggagagggacaaggccgccggcctgatccccttcttcatggtggccaccctgggcaccaccacctgctgcagcttcgacaacctgctggaggtgggccccatctgcaacaaggaggacatctggctgcacgtggacgccgcctacgccggcagcgccttcatctgccccgagttcaggcacctgctgaacggcgtggagttcgccgacagcttcaacttcaacccccacaagtggctgctggtgaacttcgactgcagcgccatgtgggtgaagaagaggaccgacctgaccggcgccttcaggctggaccccacctacctgaagcacagccaccaggacagcggcctgatcaccgactacaggcactggcagatccccctgggcaggaggttcaggagcctgaagatgtggttcgtgttcaggatgtacggcgtgaagggcctgcaggcctacatcaggaagcacgtgcagctgagccacgagttcgagagcctggtgaggcaggaccccaggttcgagatctgcgtggaggtgatcctgggcctggtgtgcttcaggctgaagggcagcaacaaggtgaacgaggccctgctgcagaggatcaacagcgccaagaagatccacctggtgccctgccacctgagggacaagttcgtgctgaggttcgccatctgcagcaggaccgtggagagcgcccacgtgcagagggcctgggagcacatcaaggagctggccgccgacgtgctgagggccgagagggagtgactcgaggggtggcatccctgtgacccctccccagtgcctctcctggccctggaagttgccactccagtgcccaccagccttgtcctaataaaattaagttgcatcattttgtctgactaggtgtccttctataatattatggggtggaggggggtggtatggagcaaggggcaagttgggaagacaacctgtagggcctgcggggtctattgggaaccaagctggagtgcagtggcacaatcttggctcactgcaatctccgcctcctgggttcaagcgattctcctgcctcagcctcccgagttgttgggattccaggcatgcatgaccaggctcagctaatttttgtttttttggtagagacggggtttcaccatattggccaggctggtctccaactcctaatctcaggtgatctacccaccttggcctcccaaattgctgggattacaggcgtgaaccactgctcccttccctgtccttcggaccgagcggcagatctaggaacccctagtgatggagttggccactccctctctgcgcgctcgctcgctcactgaggccgggcgaccaaaggtcgcccgacgcccgggctttgcccgggcggcctcagtgagcgagcgagcgcgcagctgcctgcagg

SEQ ID NO: 14 - DNA, 2709 bp, synthetic construct
  source 1..2709: mol_type = other DNA; note = HRPDAAV01-B
cctgcaggcagctgcgcgctcgctcgctcactgaggccgcccgggcaaagcccgggcgtcgggcgacctttggtcgcccggcctcagtgagcgagcgagcgcgcagagagggagtggccaactccatcactaggggttcctatcgatatcaagcttcgttacataacttacggtaaatggcccgcctggctgaccgcccaacgacccccgcccattgacgtcaatagtaacgccaatagggactttccattgacgtcaatgggtggagtatttacggtaaactgcccacttggcagtacatcaagtgtatcatatgccaagtacgccccctattgacgtcaatgacggtaaatggcccgcctggcattgtgcccagtacatgaccttatgggactttcctacttggcagtacatctacgtattagtcatcgctattaccatggtcgaggtgagccccacgttctgcttcactctccccatctcccccccctccccacccccaattttgtatttatttattttttaattattttgtgcagcgatgggggcggggggggggggggggcgcgcgccaggcggggcggggcggggcgaggggcggggcggggcgaggcggagaggtgcggcggcagccaatcagagcggcgcgctccgaaagtttccttttatggcgaggcggcggcggcggcggccctataaaaagcgaagcgcgcggcgggcgggagtcgctgcgcgctgccttcgccccgtgccccgctccgccgccgcctcgcgccgcccgccccggctctgactgaccgcgttactcccacaggtgagcgggcgggacggcccttctcctccgggctgtaattagctgagcaagaggtaagggtttaagggatggttggttggtggggtattaatgtttaattacctggagcacctgcctgaaatcactttttttcaggttgggggattcgaacatcggccgccaccatgaacgccagcgagttcaggaggaggggcaaggagatggtggactacgtggccaactacatggagggcatcgagggcaggcaggtgtaccccgacgtggagcccggctacctgaggcccctgatccccgccgccgccccccaggagcccgacaccttcgaggacatcatcaacgacgtggagaagatcatcatgcccggcgtgacccactggcacagcccctacttcttcgcctacttccccaccgccagcagctaccccgccatgctggccgacatgctgtgcggcgccatcggctgcatcggcttcagctgggccgccagccccgcctgcaccgagctggagaccgtgatgatggactggctgggcaagatgctggagctgcccaaggccttcctgaacgagaaggccggcgagggcggcggcgtgatccagggcagcgccagcgaggccaccctggtggccctgctggccgccaggaccaaggtgatccacaggctgcaggccgccagccccgagctgacccaggccgccatcatggagaagctggtggcctacagcagcgaccaggcccacagcagcgtggagagggccggcctgatcggcggcgtgaagctgaaggccatccccagcgacggcaacttcgccatgagggccagcgccctgcaggaggccctggagagggacaaggccgccggcctgatccccttcttcatggtggccaccctgggcaccaccacctgctgcagcttcgacaacctgctggaggtgggccccatctgcaacaaggaggacatctggctgcacgtggacgccgcctacgccggcagcgccttcatctgccccgagttcaggcacctgctgaacggcgtggagttcgccgacagcttcaacttcaacccccacaagtggctgctggtgaacttcgactgcagcgccatgtgggtgaagaagaggaccgacctgaccggcgccttcaggctggaccccacctacctgaagcacagccaccaggacagcggcctgatcaccgactacaggcactggcagatccccctgggcaggaggttcaggagcctgaagatgtggttcgtgttcaggatgtacggcgtgaagggcctgcaggcctacatcaggaagcacgtgcagctgagccacgagttcgagagcctggtgaggcaggaccccaggttcgagatctgcgtggaggtgatcctgggcctggtgtgcttcaggctgaagggcagcaacaaggtgaacgaggccctgctgcagaggatcaacagcgccaagaagatccacctggtgccctgccacctgagggacaagttcgtgctgaggttcgccatctgcagcaggaccgtggagagcgcccacgtgcagagggcctgggagcacatcaaggagctggccgccgacgtgctgagggccgagagggagtgactcgagtaagatacattgatgagtttggacaaaccacaactagaatgcagtgaaaaaaatgctttatttgtgaaatttgtgatgctattgctttatttgtaaccattataagctgcaataaacaagttcggaccgagcggcagatctaggaacccctagtgatggagttggccactccctctctgcgcgctcgctcgctcactgaggccgggcgaccaaaggtcgcccgacgcccgggctttgcccgggcggcctcagtgagcgagcgagcgcgcagctgcctgcagg

SEQ ID NO: 15 - DNA, 3298 bp, synthetic construct
  source 1..3298: mol_type = other DNA; note = HRPDAAV01-C
cctgcaggcagctgcgcgctcgctcgctcactgaggccgcccgggcaaagcccgggcgtcgggcgacctttggtcgcccggcctcagtgagcgagcgagcgcgcagagagggagtggccaactccatcactaggggttcctatcgatatcaagcttcgttacataacttacggtaaatggcccgcctggctgaccgcccaacgacccccgcccattgacgtcaatagtaacgccaatagggactttccattgacgtcaatgggtggagtatttacggtaaactgcccacttggcagtacatcaagtgtatcatatgccaagtacgccccctattgacgtcaatgacggtaaatggcccgcctggcattgtgcccagtacatgaccttatgggactttcctacttggcagtacatctacgtattagtcatcgctattaccatggtcgaggtgagccccacgttctgcttcactctccccatctcccccccctccccacccccaattttgtatttatttattttttaattattttgtgcagcgatgggggcggggggggggggggggcgcgcgccaggcggggcggggcggggcgaggggcggggcggggcgaggcggagaggtgcggcggcagccaatcagagcggcgcgctccgaaagtttccttttatggcgaggcggcggcggcggcggccctataaaaagcgaagcgcgcggcgggcgggagtcgctgcgcgctgccttcgccccgtgccccgctccgccgccgcctcgcgccgcccgccccggctctgactgaccgcgttactcccacaggtgagcgggcgggacggcccttctcctccgggctgtaattagctgagcaagaggtaagggtttaagggatggttggttggtggggtattaatgtttaattacctggagcacctgcctgaaatcactttttttcaggttgggggattcgaacatcggccgccaccatgaacgccagcgagttcaggaggaggggcaaggagatggtggactacgtggccaactacatggagggcatcgagggcaggcaggtgtaccccgacgtggagcccggctacctgaggcccctgatccccgccgccgccccccaggagcccgacaccttcgaggacatcatcaacgacgtggagaagatcatcatgcccggcgtgacccactggcacagcccctacttcttcgcctacttccccaccgccagcagctaccccgccatgctggccgacatgctgtgcggcgccatcggctgcatcggcttcagctgggccgccagccccgcctgcaccgagctggagaccgtgatgatggactggctgggcaagatgctggagctgcccaaggccttcctgaacgagaaggccggcgagggcggcggcgtgatccagggcagcgccagcgaggccaccctggtggccctgctggccgccaggaccaaggtgatccacaggctgcaggccgccagccccgagctgacccaggccgccatcatggagaagctggtggcctacagcagcgaccaggcccacagcagcgtggagagggccggcctgatcggcggcgtgaagctgaaggccatccccagcgacggcaacttcgccatgagggccagcgccctgcaggaggccctggagagggacaaggccgccggcctgatccccttcttcatggtggccaccctgggcaccaccacctgctgcagcttcgacaacctgctggaggtgggccccatctgcaacaaggaggacatctggctgcacgtggacgccgcctacgccggcagcgccttcatctgccccgagttcaggcacctgctgaacggcgtggagttcgccgacagcttcaacttcaacccccacaagtggctgctggtgaacttcgactgcagcgccatgtgggtgaagaagaggaccgacctgaccggcgccttcaggctggaccccacctacctgaagcacagccaccaggacagcggcctgatcaccgactacaggcactggcagatccccctgggcaggaggttcaggagcctgaagatgtggttcgtgttcaggatgtacggcgtgaagggcctgcaggcctacatcaggaagcacgtgcagctgagccacgagttcgagagcctggtgaggcaggaccccaggttcgagatctgcgtggaggtgatcctgggcctggtgtgcttcaggctgaagggcagcaacaaggtgaacgaggccctgctgcagaggatcaacagcgccaagaagatccacctggtgccctgccacctgagggacaagttcgtgctgaggttcgccatctgcagcaggaccgtggagagcgcccacgtgcagagggcctgggagcacatcaaggagctggccgccgacgtgctgagggccgagagggagtgactcgagaatcaacctctggattacaaaatttgtgaaagattgactggtattcttaactatgttgctccttttacgctatgtggatacgctgctttaatgcctttgtatcatgctattgcttcccgtatggctttcattttctcctccttgtataaatcctggttgctgtctctttatgaggagttgtggcccgttgtcaggcaacgtggcgtggtgtgcactgtgtttgctgacgcaacccccactggttggggcattgccaccacctgtcagctcctttccgggactttcgctttccccctccctattgccacggcggaactcatcgccgcctgccttgcccgctgctggacaggggctcggctgttgggcactgacaattccgtggtgttgtcggggaaatcatcgtcctttccttggctgctcgcctgtgttgccacctggattctgcgcgggacgtccttctgctacgtcccttcggccctcaatccagcggaccttccttcccgcggcctgctgccggctctgcggcctcttccgcgtcttcgccttcgccctcagacgagtcggatctccctttgggccgcctccccgctaagatacattgatgagtttggacaaaccacaactagaatgcagtgaaaaaaatgctttatttgtgaaatttgtgatgctattgctttatttgtaaccattataagctgcaataaacaagttcggaccgagcggcagatctaggaacccctagtgatggagttggccactccctctctgcgcgctcgctcgctcactgaggccgggcgaccaaaggtcgcccgacgcccgggctttgcccgggcggcctcagtgagcgagcgagcgcgcagctgcctgcagg

SEQ ID NO: 16 - DNA, 3988 bp, synthetic construct
  source 1..3988: mol_type = other DNA; note = HRPDAAV02-A
cctgcaggcagctgcgcgctcgctcgctcactgaggccgcccgggcaaagcccgggcgtcgggcgacctttggtcgcccggcctcagtgagcgagcgagcgcgcagagagggagtggccaactccatcactaggggttcctatcgatatcaagcttcgttacataacttacggtaaatggcccgcctggctgaccgcccaacgacccccgcccattgacgtcaatagtaacgccaatagggactttccattgacgtcaatgggtggagtatttacggtaaactgcccacttggcagtacatcaagtgtatcatatgccaagtacgccccctattgacgtcaatgacggtaaatggcccgcctggcattgtgcccagtacatgaccttatgggactttcctacttggcagtacatctacgtattagtcatcgctattaccatggtcgaggtgagccccacgttctgcttcactctccccatctcccccccctccccacccccaattttgtatttatttattttttaattattttgtgcagcgatgggggcggggggggggggggggcgcgcgccaggcggggcggggcggggcgaggggcggggcggggcgaggcggagaggtgcggcggcagccaatcagagcggcgcgctccgaaagtttccttttatggcgaggcggcggcggcggcggccctataaaaagcgaagcgcgcggcgggcgggagtcgctgcgcgctgccttcgccccgtgccccgctccgccgccgcctcgcgccgcccgccccggctctgactgaccgcgttactcccacaggtgagcgggcgggacggcccttctcctccgggctgtaattagctgagcaagaggtaagggtttaagggatggttggttggtggggtattaatgtttaattacctggagcacctgcctgaaatcactttttttcaggttgggggattcgaacatcggccgccaccatgaacgccagcgagttcaggaggaggggcaaggagatggtggactacgtggccaactacatggagggcatcgagggcaggcaggtgtaccccgacgtggagcccggctacctgaggcccctgatccccgccgccgccccccaggagcccgacaccttcgaggacatcatcaacgacgtggagaagatcatcatgcccggcgtgacccactggcacagcccctacttcttcgcctacttccccaccgccagcagctaccccgccatgctggccgacatgctgtgcggcgccatcggctgcatcggcttcagctgggccgccagccccgcctgcaccgagctggagaccgtgatgatggactggctgggcaagatgctggagctgcccaaggccttcctgaacgagaaggccggcgagggcggcggcgtgatccagggcagcgccagcgaggccaccctggtggccctgctggccgccaggaccaaggtgatccacaggctgcaggccgccagccccgagctgacccaggccgccatcatggagaagctggtggcctacagcagcgaccaggcccacagcagcgtggagagggccggcctgatcggcggcgtgaagctgaaggccatccccagcgacggcaacttcgccatgagggccagcgccctgcaggaggccctggagagggacaaggccgccggcctgatccccttcttcatggtggccaccctgggcaccaccacctgctgcagcttcgacaacctgctggaggtgggccccatctgcaacaaggaggacatctggctgcacgtggacgccgcctacgccggcagcgccttcatctgccccgagttcaggcacctgctgaacggcgtggagttcgccgacagcttcaacttcaacccccacaagtggctgctggtgaacttcgactgcagcgccatgtgggtgaagaagaggaccgacctgaccggcgccttcaggctggaccccacctacctgaagcacagccaccaggacagcggcctgatcaccgactacaggcactggcagatccccctgggcaggaggttcaggagcctgaagatgtggttcgtgttcaggatgtacggcgtgaagggcctgcaggcctacatcaggaagcacgtgcagctgagccacgagttcgagagcctggtgaggcaggaccccaggttcgagatctgcgtggaggtgatcctgggcctggtgtgcttcaggctgaagggcagcaacaaggtgaacgaggccctgctgcagaggatcaacagcgccaagaagatccacctggtgccctgccacctgagggacaagttcgtgctgaggttcgccatctgcagcaggaccgtggagagcgcccacgtgcagagggcctgggagcacatcaaggagctggccgccgacgtgctgagggccgagagggaggccaccaacttctccctgctgaagcaggccggcgacgtggaggagaaccccggccccatgaagttatgggatgtcgtggctgtctgcctggtgctgctccacaccgcgtccgccttcccgctgcccgccggtaagaggcctcccgaggcgcccgccgaagaccgctccctcggccgccgccgcgcgcccttcgcgctgagcagtgactcaaatatgccagaggattatcctgatcagttcgatgatgtcatggattttattcaagccaccattaaaagactgaaaaggtcaccagataaacaaatggcagtgcttcctagaagagagcggaatcggcaggctgcagctgccaacccagagaattccagaggaaaaggtcggagaggccagaggggcaaaaaccggggttgtgtcttaactgcaatacatttaaatgtcactgacttgggtctgggctatgaaaccaaggaggaactgatttttaggtactgcagcggctcttgcgatgcagctgagacaacgtacgacaaaatattgaaaaacttatccagaaatagaaggctggtgagtgacaaagtagggcaggcatgttgcagacccatcgcctttgatgatgacctgtcgtttttagatgataacctggtttaccatattctaagaaagcattccgctaaaaggtgtggatgtatctgactcgagaatcaacctctggattacaaaatttgtgaaagattgactggtattcttaactatgttgctccttttacgctatgtggatacgctgctttaatgcctttgtatcatgctattgcttcccgtatggctttcattttctcctccttgtataaatcctggttgctgtctctttatgaggagttgtggcccgttgtcaggcaacgtggcgtggtgtgcactgtgtttgctgacgcaacccccactggttggggcattgccaccacctgtcagctcctttccgggactttcgctttccccctccctattgccacggcggaactcatcgccgcctgccttgcccgctgctggacaggggctcggctgttgggcactgacaattccgtggtgttgtcggggaaatcatcgtcctttccttggctgctcgcctgtgttgccacctggattctgcgcgggacgtccttctgctacgtcccttcggccctcaatccagcggaccttccttcccgcggcctgctgccggctctgcggcctcttccgcgtcttcgccttcgccctcagacgagtcggatctccctttgggccgcctccccgctaagatacattgatgagtttggacaaaccacaactagaatgcagtgaaaaaaatgctttatttgtgaaatttgtgatgctattgctttatttgtaaccattataagctgcaataaacaagttcggaccgagcggcagatctaggaacccctagtgatggagttggccactccctctctgcgcgctcgctcgctcactgaggccgggcgaccaaaggtcgcccgacgcccgggctttgcccgggcggcctcagtgagcgagcgagcgcgcagctgcctgcagg

SEQ ID NO: 17 - DNA, 3991 bp, synthetic construct
  source 1..3991: mol_type = other DNA; note = HRPDAAV02-B
cctgcaggcagctgcgcgctcgctcgctcactgaggccgcccgggcaaagcccgggcgtcgggcgacctttggtcgcccggcctcagtgagcgagcgagcgcgcagagagggagtggccaactccatcactaggggttcctatcgatatcaagcttcgttacataacttacggtaaatggcccgcctggctgaccgcccaacgacccccgcccattgacgtcaatagtaacgccaatagggactttccattgacgtcaatgggtggagtatttacggtaaactgcccacttggcagtacatcaagtgtatcatatgccaagtacgccccctattgacgtcaatgacggtaaatggcccgcctggcattgtgcccagtacatgaccttatgggactttcctacttggcagtacatctacgtattagtcatcgctattaccatggtcgaggtgagccccacgttctgcttcactctccccatctcccccccctccccacccccaattttgtatttatttattttttaattattttgtgcagcgatgggggcggggggggggggggggcgcgcgccaggcggggcggggcggggcgaggggcggggcggggcgaggcggagaggtgcggcggcagccaatcagagcggcgcgctccgaaagtttccttttatggcgaggcggcggcggcggcggccctataaaaagcgaagcgcgcggcgggcgggagtcgctgcgcgctgccttcgccccgtgccccgctccgccgccgcctcgcgccgcccgccccggctctgactgaccgcgttactcccacaggtgagcgggcgggacggcccttctcctccgggctgtaattagctgagcaagaggtaagggtttaagggatggttggttggtggggtattaatgtttaattacctggagcacctgcctgaaatcactttttttcaggttgggggattcgaacatcggccgccaccatgaagttatgggatgtcgtggctgtctgcctggtgctgctccacaccgcgtccgccttcccgctgcccgccggtaagaggcctcccgaggcgcccgccgaagaccgctccctcggccgccgccgcgcgcccttcgcgctgagcagtgactcaaatatgccagaggattatcctgatcagttcgatgatgtcatggattttattcaagccaccattaaaagactgaaaaggtcaccagataaacaaatggcagtgcttcctagaagagagcggaatcggcaggctgcagctgccaacccagagaattccagaggaaaaggtcggagaggccagaggggcaaaaaccggggttgtgtcttaactgcaatacatttaaatgtcactgacttgggtctgggctatgaaaccaaggaggaactgatttttaggtactgcagcggctcttgcgatgcagctgagacaacgtacgacaaaatattgaaaaacttatccagaaatagaaggctggtgagtgacaaagtagggcaggcatgttgcagacccatcgcctttgatgatgacctgtcgtttttagatgataacctggtttaccatattctaagaaagcattccgctaaaaggtgtggatgtatctgagccaccaacttctccctgctgaagcaggccggcgacgtggaggagaaccccggccccatgaacgccagcgagttcaggaggaggggcaaggagatggtggactacgtggccaactacatggagggcatcgagggcaggcaggtgtaccccgacgtggagcccggctacctgaggcccctgatccccgccgccgccccccaggagcccgacaccttcgaggacatcatcaacgacgtggagaagatcatcatgcccggcgtgacccactggcacagcccctacttcttcgcctacttccccaccgccagcagctaccccgccatgctggccgacatgctgtgcggcgccatcggctgcatcggcttcagctgggccgccagccccgcctgcaccgagctggagaccgtgatgatggactggctgggcaagatgctggagctgcccaaggccttcctgaacgagaaggccggcgagggcggcggcgtgatccagggcagcgccagcgaggccaccctggtggccctgctggccgccaggaccaaggtgatccacaggctgcaggccgccagccccgagctgacccaggccgccatcatggagaagctggtggcctacagcagcgaccaggcccacagcagcgtggagagggccggcctgatcggcggcgtgaagctgaaggccatccccagcgacggcaacttcgccatgagggccagcgccctgcaggaggccctggagagggacaaggccgccggcctgatccccttcttcatggtggccaccctgggcaccaccacctgctgcagcttcgacaacctgctggaggtgggccccatctgcaacaaggaggacatctggctgcacgtggacgccgcctacgccggcagcgccttcatctgccccgagttcaggcacctgctgaacggcgtggagttcgccgacagcttcaacttcaacccccacaagtggctgctggtgaacttcgactgcagcgccatgtgggtgaagaagaggaccgacctgaccggcgccttcaggctggaccccacctacctgaagcacagccaccaggacagcggcctgatcaccgactacaggcactggcagatccccctgggcaggaggttcaggagcctgaagatgtggttcgtgttcaggatgtacggcgtgaagggcctgcaggcctacatcaggaagcacgtgcagctgagccacgagttcgagagcctggtgaggcaggaccccaggttcgagatctgcgtggaggtgatcctgggcctggtgtgcttcaggctgaagggcagcaacaaggtgaacgaggccctgctgcagaggatcaacagcgccaagaagatccacctggtgccctgccacctgagggacaagttcgtgctgaggttcgccatctgcagcaggaccgtggagagcgcccacgtgcagagggcctgggagcacatcaaggagctggccgccgacgtgctgagggccgagagggagtgactcgagaatcaacctctggattacaaaatttgtgaaagattgactggtattcttaactatgttgctccttttacgctatgtggatacgctgctttaatgcctttgtatcatgctattgcttcccgtatggctttcattttctcctccttgtataaatcctggttgctgtctctttatgaggagttgtggcccgttgtcaggcaacgtggcgtggtgtgcactgtgtttgctgacgcaacccccactggttggggcattgccaccacctgtcagctcctttccgggactttcgctttccccctccctattgccacggcggaactcatcgccgcctgccttgcccgctgctggacaggggctcggctgttgggcactgacaattccgtggtgttgtcggggaaatcatcgtcctttccttggctgctcgcctgtgttgccacctggattctgcgcgggacgtccttctgctacgtcccttcggccctcaatccagcggaccttccttcccgcggcctgctgccggctctgcggcctcttccgcgtcttcgccttcgccctcagacgagtcggatctccctttgggccgcctccccgctaagatacattgatgagtttggacaaaccacaactagaatgcagtgaaaaaaatgctttatttgtgaaatttgtgatgctattgctttatttgtaaccattataagctgcaataaacaagttcggaccgagcggcagatctaggaacccctagtgatggagttggccactccctctctgcgcgctcgctcgctcactgaggccgggcgaccaaaggtcgcccgacgcccgggctttgcccgggcggcctcagtgagcgagcgagcgcgcagctgcctgcagg

SEQ ID NO: 18 - DNA, 3933 bp, synthetic construct
  source 1..3933: mol_type = other DNA; note = HRPDAAV03-A
cctgcaggcagctgcgcgctcgctcgctcactgaggccgcccgggcaaagcccgggcgtcgggcgacctttggtcgcccggcctcagtgagcgagcgagcgcgcagagagggagtggccaactccatcactaggggttcctatcgatatcaagcttcgttacataacttacggtaaatggcccgcctggctgaccgcccaacgacccccgcccattgacgtcaatagtaacgccaatagggactttccattgacgtcaatgggtggagtatttacggtaaactgcccacttggcagtacatcaagtgtatcatatgccaagtacgccccctattgacgtcaatgacggtaaatggcccgcctggcattgtgcccagtacatgaccttatgggactttcctacttggcagtacatctacgtattagtcatcgctattaccatggtcgaggtgagccccacgttctgcttcactctccccatctcccccccctccccacccccaattttgtatttatttattttttaattattttgtgcagcgatgggggcggggggggggggggggcgcgcgccaggcggggcggggcggggcgaggggcggggcggggcgaggcggagaggtgcggcggcagccaatcagagcggcgcgctccgaaagtttccttttatggcgaggcggcggcggcggcggccctataaaaagcgaagcgcgcggcgggcgggagtcgctgcgcgctgccttcgccccgtgccccgctccgccgccgcctcgcgccgcccgccccggctctgactgaccgcgttactcccacaggtgagcgggcgggacggcccttctcctccgggctgtaattagctgagcaagaggtaagggtttaagggatggttggttggtggggtattaatgtttaattacctggagcacctgcctgaaatcactttttttcaggttgggggattcgaacatcggccgccaccatgaacgccagcgagttcaggaggaggggcaaggagatggtggactacgtggccaactacatggagggcatcgagggcaggcaggtgtaccccgacgtggagcccggctacctgaggcccctgatccccgccgccgccccccaggagcccgacaccttcgaggacatcatcaacgacgtggagaagatcatcatgcccggcgtgacccactggcacagcccctacttcttcgcctacttccccaccgccagcagctaccccgccatgctggccgacatgctgtgcggcgccatcggctgcatcggcttcagctgggccgccagccccgcctgcaccgagctggagaccgtgatgatggactggctgggcaagatgctggagctgcccaaggccttcctgaacgagaaggccggcgagggcggcggcgtgatccagggcagcgccagcgaggccaccctggtggccctgctggccgccaggaccaaggtgatccacaggctgcaggccgccagccccgagctgacccaggccgccatcatggagaagctggtggcctacagcagcgaccaggcccacagcagcgtggagagggccggcctgatcggcggcgtgaagctgaaggccatccccagcgacggcaacttcgccatgagggccagcgccctgcaggaggccctggagagggacaaggccgccggcctgatccccttcttcatggtggccaccctgggcaccaccacctgctgcagcttcgacaacctgctggaggtgggccccatctgcaacaaggaggacatctggctgcacgtggacgccgcctacgccggcagcgccttcatctgccccgagttcaggcacctgctgaacggcgtggagttcgccgacagcttcaacttcaacccccacaagtggctgctggtgaacttcgactgcagcgccatgtgggtgaagaagaggaccgacctgaccggcgccttcaggctggaccccacctacctgaagcacagccaccaggacagcggcctgatcaccgactacaggcactggcagatccccctgggcaggaggttcaggagcctgaagatgtggttcgtgttcaggatgtacggcgtgaagggcctgcaggcctacatcaggaagcacgtgcagctgagccacgagttcgagagcctggtgaggcaggaccccaggttcgagatctgcgtggaggtgatcctgggcctggtgtgcttcaggctgaagggcagcaacaaggtgaacgaggccctgctgcagaggatcaacagcgccaagaagatccacctggtgccctgccacctgagggacaagttcgtgctgaggttcgccatctgcagcaggaccgtggagagcgcccacgtgcagagggcctgggagcacatcaaggagctggccgccgacgtgctgagggccgagagggagtgactcgagtaagatacattgatgagtttggacaaaccacaactagaatgcagtgaaaaaaatgctttatttgtgaaatttgtgatgctattgctttatttgtaaccattataagctgcaataaacaagttcgttacataacttacggtaaatggcccgcctggctgaccgcccaacgacccccgcccattgacgtcaataatgacgtatgttcccatagtaacgtcaatagggactttccattgacgtcaatgggtggagtatttacggtaaactgcccacttggcagtacatcaagtgtatcatatgccaagtacgccccctattgacgtcaatgacggtaaatggcccgcctggcattatgcccagtacatgaccttatgggactttcctacttggcagtacatctacgtattagtcatcgctattaccatggtgatgcggttttggcagtacatcaatgggcgtggatagcggtttgactcacggggatttccaagtctccaccccattgacgtcaatgggagtttgttttgcaccaaaatcaacgggactttccaaaatgtcgtaacaactccgccccattgacgcaaatgggcggtaggcgtgtacggtgggaggtctatataagcagagctgccaccatgaagttatgggatgtcgtggctgtctgcctggtgctgctccacaccgcgtccgccttcccgctgcccgccggtaagaggcctcccgaggcgcccgccgaagaccgctccctcggccgccgccgcgcgcccttcgcgctgagcagtgactcaaatatgccagaggattatcctgatcagttcgatgatgtcatggattttattcaagccaccattaaaagactgaaaaggtcaccagataaacaaatggcagtgcttcctagaagagagcggaatcggcaggctgcagctgccaacccagagaattccagaggaaaaggtcggagaggccagaggggcaaaaaccggggttgtgtcttaactgcaatacatttaaatgtcactgacttgggtctgggctatgaaaccaaggaggaactgatttttaggtactgcagcggctcttgcgatgcagctgagacaacgtacgacaaaatattgaaaaacttatccagaaatagaaggctggtgagtgacaaagtagggcaggcatgttgcagacccatcgcctttgatgatgacctgtcgtttttagatgataacctggtttaccatattctaagaaagcattccgctaaaaggtgtggatgtatctgaaataaagtctgagtgggcggcagcctgtgtgtgcctgggttctctctgtcccggaatgtgcaaacaatggaggtgcggaccgagcggcagatctaggaacccctagtgatggagttggccactccctctctgcgcgctcgctcgctcactgaggccgggcgaccaaaggtcgcccgacgcccgggctttgcccgggcggcctcagtgagcgagcgagcgcgcagctgcctgcagg

SEQ ID NO: 19 - DNA, 4522 bp, synthetic construct
  source 1..4522: mol_type = other DNA; note = HRPDAAV03-B
cctgcaggcagctgcgcgctcgctcgctcactgaggccgcccgggcaaagcccgggcgtcgggcgacctttggtcgcccggcctcagtgagcgagcgagcgcgcagagagggagtggccaactccatcactaggggttcctatcgatatcaagcttcgttacataacttacggtaaatggcccgcctggctgaccgcccaacgacccccgcccattgacgtcaatagtaacgccaatagggactttccattgacgtcaatgggtggagtatttacggtaaactgcccacttggcagtacatcaagtgtatcatatgccaagtacgccccctattgacgtcaatgacggtaaatggcccgcctggcattgtgcccagtacatgaccttatgggactttcctacttggcagtacatctacgtattagtcatcgctattaccatggtcgaggtgagccccacgttctgcttcactctccccatctcccccccctccccacccccaattttgtatttatttattttttaattattttgtgcagcgatgggggcggggggggggggggggcgcgcgccaggcggggcggggcggggcgaggggcggggcggggcgaggcggagaggtgcggcggcagccaatcagagcggcgcgctccgaaagtttccttttatggcgaggcggcggcggcggcggccctataaaaagcgaagcgcgcggcgggcgggagtcgctgcgcgctgccttcgccccgtgccccgctccgccgccgcctcgcgccgcccgccccggctctgactgaccgcgttactcccacaggtgagcgggcgggacggcccttctcctccgggctgtaattagctgagcaagaggtaagggtttaagggatggttggttggtggggtattaatgtttaattacctggagcacctgcctgaaatcactttttttcaggttgggggattcgaacatcggccgccaccatgaacgccagcgagttcaggaggaggggcaaggagatggtggactacgtggccaactacatggagggcatcgagggcaggcaggtgtaccccgacgtggagcccggctacctgaggcccctgatccccgccgccgccccccaggagcccgacaccttcgaggacatcatcaacgacgtggagaagatcatcatgcccggcgtgacccactggcacagcccctacttcttcgcctacttccccaccgccagcagctaccccgccatgctggccgacatgctgtgcggcgccatcggctgcatcggcttcagctgggccgccagccccgcctgcaccgagctggagaccgtgatgatggactggctgggcaagatgctggagctgcccaaggccttcctgaacgagaaggccggcgagggcggcggcgtgatccagggcagcgccagcgaggccaccctggtggccctgctggccgccaggaccaaggtgatccacaggctgcaggccgccagccccgagctgacccaggccgccatcatggagaagctggtggcctacagcagcgaccaggcccacagcagcgtggagagggccggcctgatcggcggcgtgaagctgaaggccatccccagcgacggcaacttcgccatgagggccagcgccctgcaggaggccctggagagggacaaggccgccggcctgatccccttcttcatggtggccaccctgggcaccaccacctgctgcagcttcgacaacctgctggaggtgggccccatctgcaacaaggaggacatctggctgcacgtggacgccgcctacgccggcagcgccttcatctgccccgagttcaggcacctgctgaacggcgtggagttcgccgacagcttcaacttcaacccccacaagtggctgctggtgaacttcgactgcagcgccatgtgggtgaagaagaggaccgacctgaccggcgccttcaggctggaccccacctacctgaagcacagccaccaggacagcggcctgatcaccgactacaggcactggcagatccccctgggcaggaggttcaggagcctgaagatgtggttcgtgttcaggatgtacggcgtgaagggcctgcaggcctacatcaggaagcacgtgcagctgagccacgagttcgagagcctggtgaggcaggaccccaggttcgagatctgcgtggaggtgatcctgggcctggtgtgcttcaggctgaagggcagcaacaaggtgaacgaggccctgctgcagaggatcaacagcgccaagaagatccacctggtgccctgccacctgagggacaagttcgtgctgaggttcgccatctgcagcaggaccgtggagagcgcccacgtgcagagggcctgggagcacatcaaggagctggccgccgacgtgctgagggccgagagggagtgactcgagtaagatacattgatgagtttggacaaaccacaactagaatgcagtgaaaaaaatgctttatttgtgaaatttgtgatgctattgctttatttgtaaccattataagctgcaataaacaagttcgttacataacttacggtaaatggcccgcctggctgaccgcccaacgacccccgcccattgacgtcaataatgacgtatgttcccatagtaacgtcaatagggactttccattgacgtcaatgggtggagtatttacggtaaactgcccacttggcagtacatcaagtgtatcatatgccaagtacgccccctattgacgtcaatgacggtaaatggcccgcctggcattatgcccagtacatgaccttatgggactttcctacttggcagtacatctacgtattagtcatcgctattaccatggtgatgcggttttggcagtacatcaatgggcgtggatagcggtttgactcacggggatttccaagtctccaccccattgacgtcaatgggagtttgttttgcaccaaaatcaacgggactttccaaaatgtcgtaacaactccgccccattgacgcaaatgggcggtaggcgtgtacggtgggaggtctatataagcagagctgccaccatgaagttatgggatgtcgtggctgtctgcctggtgctgctccacaccgcgtccgccttcccgctgcccgccggtaagaggcctcccgaggcgcccgccgaagaccgctccctcggccgccgccgcgcgcccttcgcgctgagcagtgactcaaatatgccagaggattatcctgatcagttcgatgatgtcatggattttattcaagccaccattaaaagactgaaaaggtcaccagataaacaaatggcagtgcttcctagaagagagcggaatcggcaggctgcagctgccaacccagagaattccagaggaaaaggtcggagaggccagaggggcaaaaaccggggttgtgtcttaactgcaatacatttaaatgtcactgacttgggtctgggctatgaaaccaaggaggaactgatttttaggtactgcagcggctcttgcgatgcagctgagacaacgtacgacaaaatattgaaaaacttatccagaaatagaaggctggtgagtgacaaagtagggcaggcatgttgcagacccatcgcctttgatgatgacctgtcgtttttagatgataacctggtttaccatattctaagaaagcattccgctaaaaggtgtggatgtatctgaaatcaacctctggattacaaaatttgtgaaagattgactggtattcttaactatgttgctccttttacgctatgtggatacgctgctttaatgcctttgtatcatgctattgcttcccgtatggctttcattttctcctccttgtataaatcctggttgctgtctctttatgaggagttgtggcccgttgtcaggcaacgtggcgtggtgtgcactgtgtttgctgacgcaacccccactggttggggcattgccaccacctgtcagctcctttccgggactttcgctttccccctccctattgccacggcggaactcatcgccgcctgccttgcccgctgctggacaggggctcggctgttgggcactgacaattccgtggtgttgtcggggaaatcatcgtcctttccttggctgctcgcctgtgttgccacctggattctgcgcgggacgtccttctgctacgtcccttcggccctcaatccagcggaccttccttcccgcggcctgctgccggctctgcggcctcttccgcgtcttcgccttcgccctcagacgagtcggatctccctttgggccgcctccccgcaataaagtctgagtgggcggcagcctgtgtgtgcctgggttctctctgtcccggaatgtgcaaacaatggaggtgcggaccgagcggcagatctaggaacccctagtgatggagttggccactccctctctgcgcgctcgctcgctcactgaggccgggcgaccaaaggtcgcccgacgcccgggctttgcccgggcggcctcagtgagcgagcgagcgcgcagctgcctgcagg

SEQ ID NO: 20 - DNA, 4506 bp, synthetic construct
  source 1..4506: mol_type = other DNA; note = HRPDAAV03-C
cctgcaggcagctgcgcgctcgctcgctcactgaggccgcccgggcaaagcccgggcgtcgggcgacctttggtcgcccggcctcagtgagcgagcgagcgcgcagagagggagtggccaactccatcactaggggttcctatcgatatcaagcttcgttacataacttacggtaaatggcccgcctggctgaccgcccaacgacccccgcccattgacgtcaatagtaacgccaatagggactttccattgacgtcaatgggtggagtatttacggtaaactgcccacttggcagtacatcaagtgtatcatatgccaagtacgccccctattgacgtcaatgacggtaaatggcccgcctggcattgtgcccagtacatgaccttatgggactttcctacttggcagtacatctacgtattagtcatcgctattaccatggtcgaggtgagccccacgttctgcttcactctccccatctcccccccctccccacccccaattttgtatttatttattttttaattattttgtgcagcgatgggggcggggggggggggggggcgcgcgccaggcggggcggggcggggcgaggggcggggcggggcgaggcggagaggtgcggcggcagccaatcagagcggcgcgctccgaaagtttccttttatggcgaggcggcggcggcggcggccctataaaaagcgaagcgcgcggcgggcgggagtcgctgcgcgctgccttcgccccgtgccccgctccgccgccgcctcgcgccgcccgccccggctctgactgaccgcgttactcccacaggtgagcgggcgggacggcccttctcctccgggctgtaattagctgagcaagaggtaagggtttaagggatggttggttggtggggtattaatgtttaattacctggagcacctgcctgaaatcactttttttcaggttgggggattcgaacatcggccgccaccatgaacgccagcgagttcaggaggaggggcaaggagatggtggactacgtggccaactacatggagggcatcgagggcaggcaggtgtaccccgacgtggagcccggctacctgaggcccctgatccccgccgccgccccccaggagcccgacaccttcgaggacatcatcaacgacgtggagaagatcatcatgcccggcgtgacccactggcacagcccctacttcttcgcctacttccccaccgccagcagctaccccgccatgctggccgacatgctgtgcggcgccatcggctgcatcggcttcagctgggccgccagccccgcctgcaccgagctggagaccgtgatgatggactggctgggcaagatgctggagctgcccaaggccttcctgaacgagaaggccggcgagggcggcggcgtgatccagggcagcgccagcgaggccaccctggtggccctgctggccgccaggaccaaggtgatccacaggctgcaggccgccagccccgagctgacccaggccgccatcatggagaagctggtggcctacagcagcgaccaggcccacagcagcgtggagagggccggcctgatcggcggcgtgaagctgaaggccatccccagcgacggcaacttcgccatgagggccagcgccctgcaggaggccctggagagggacaaggccgccggcctgatccccttcttcatggtggccaccctgggcaccaccacctgctgcagcttcgacaacctgctggaggtgggccccatctgcaacaaggaggacatctggctgcacgtggacgccgcctacgccggcagcgccttcatctgccccgagttcaggcacctgctgaacggcgtggagttcgccgacagcttcaacttcaacccccacaagtggctgctggtgaacttcgactgcagcgccatgtgggtgaagaagaggaccgacctgaccggcgccttcaggctggaccccacctacctgaagcacagccaccaggacagcggcctgatcaccgactacaggcactggcagatccccctgggcaggaggttcaggagcctgaagatgtggttcgtgttcaggatgtacggcgtgaagggcctgcaggcctacatcaggaagcacgtgcagctgagccacgagttcgagagcctggtgaggcaggaccccaggttcgagatctgcgtggaggtgatcctgggcctggtgtgcttcaggctgaagggcagcaacaaggtgaacgaggccctgctgcagaggatcaacagcgccaagaagatccacctggtgccctgccacctgagggacaagttcgtgctgaggttcgccatctgcagcaggaccgtggagagcgcccacgtgcagagggcctgggagcacatcaaggagctggccgccgacgtgctgagggccgagagggagtgactcgagtaagatacattgatgagtttggacaaaccacaactagaatgcagtgaaaaaaatgctttatttgtgaaatttgtgatgctattgctttatttgtaaccattataagctgcaataaacaagttcgttacataacttacggtaaatggcccgcctggctgaccgcccaacgacccccgcccattgacgtcaataatgacgtatgttcccatagtaacgtcaatagggactttccattgacgtcaatgggtggagtatttacggtaaactgcccacttggcagtacatcaagtgtatcatatgccaagtacgccccctattgacgtcaatgacggtaaatggcccgcctggcattatgcccagtacatgaccttatgggactttcctacttggcagtacatctacgtattagtcatcgctattaccatggtgatgcggttttggcagtacatcaatgggcgtggatagcggtttgactcacggggatttccaagtctccaccccattgacgtcaatgggagtttgttttgcaccaaaatcaacgggactttccaaaatgtcgtaacaactccgccccattgacgcaaatgggcggtaggcgtgtacggtgggaggtctatataagcagagctgtgagtttggggacccttgattgttctttctttttcgctattgtaaaattcatgttatatggagggggcaaagttttcagggtgttgtttagaatgggaagatgtcccttgtatcaccatggaccctcatgataattttgtttctttcactttctactctgttgacaaccattgtctcctcttattttcttttcattttctgtaactttttcgttaaactttagcttgcatttgtaacgaatttttaaattcacttttgtttatttgtcagattgtaagtactttctctaatcacttttttttcaaggcaatcagggtatattatattgtacttcagcacagttttagagaacaattgttataattaaatgataaggtagaatatttctgcatataaattctggctggcgtggaaatattcttattggtagaaacaactacatcctggtcatcatcctgcctttctctttatggttacaatgatatacactgtttgagatgaggataaaatactctgagtccaaaccgggcccctctgctaaccatgttcatgccttcttctttttcctacaggccaccatgaagttatgggatgtcgtggctgtctgcctggtgctgctccacaccgcgtccgccttcccgctgcccgccggtaagaggcctcccgaggcgcccgccgaagaccgctccctcggccgccgccgcgcgcccttcgcgctgagcagtgactcaaatatgccagaggattatcctgatcagttcgatgatgtcatggattttattcaagccaccattaaaagactgaaaaggtcaccagataaacaaatggcagtgcttcctagaagagagcggaatcggcaggctgcagctgccaacccagagaattccagaggaaaaggtcggagaggccagaggggcaaaaaccggggttgtgtcttaactgcaatacatttaaatgtcactgacttgggtctgggctatgaaaccaaggaggaactgatttttaggtactgcagcggctcttgcgatgcagctgagacaacgtacgacaaaatattgaaaaacttatccagaaatagaaggctggtgagtgacaaagtagggcaggcatgttgcagacccatcgcctttgatgatgacctgtcgtttttagatgataacctggtttaccatattctaagaaagcattccgctaaaaggtgtggatgtatctgaaataaagtctgagtgggcggcagcctgtgtgtgcctgggttctctctgtcccggaatgtgcaaacaatggaggtgcggaccgagcggcagatctaggaacccctagtgatggagttggccactccctctctgcgcgctcgctcgctcactgaggccgggcgaccaaaggtcgcccgacgcccgggctttgcccgggcggcctcagtgagcgagcgagcgcgcagctgcctgcagg

SEQ ID NO: 21 - DNA, 4506 bp, synthetic construct
  source 1..4506: mol_type = other DNA; note = HRPDAAV03-D
cctgcaggcagctgcgcgctcgctcgctcactgaggccgcccgggcaaagcccgggcgtcgggcgacctttggtcgcccggcctcagtgagcgagcgagcgcgcagagagggagtggccaactccatcactaggggttcctatcgatatccgttacataacttacggtaaatggcccgcctggctgaccgcccaacgacccccgcccattgacgtcaataatgacgtatgttcccatagtaacgtcaatagggactttccattgacgtcaatgggtggagtatttacggtaaactgcccacttggcagtacatcaagtgtatcatatgccaagtacgccccctattgacgtcaatgacggtaaatggcccgcctggcattatgcccagtacatgaccttatgggactttcctacttggcagtacatctacgtattagtcatcgctattaccatggtgatgcggttttggcagtacatcaatgggcgtggatagcggtttgactcacggggatttccaagtctccaccccattgacgtcaatgggagtttgttttgcaccaaaatcaacgggactttccaaaatgtcgtaacaactccgccccattgacgcaaatgggcggtaggcgtgtacggtgggaggtctatataagcagagctgtgagtttggggacccttgattgttctttctttttcgctattgtaaaattcatgttatatggagggggcaaagttttcagggtgttgtttagaatgggaagatgtcccttgtatcaccatggaccctcatgataattttgtttctttcactttctactctgttgacaaccattgtctcctcttattttcttttcattttctgtaactttttcgttaaactttagcttgcatttgtaacgaatttttaaattcacttttgtttatttgtcagattgtaagtactttctctaatcacttttttttcaaggcaatcagggtatattatattgtacttcagcacagttttagagaacaattgttataattaaatgataaggtagaatatttctgcatataaattctggctggcgtggaaatattcttattggtagaaacaactacatcctggtcatcatcctgcctttctctttatggttacaatgatatacactgtttgagatgaggataaaatactctgagtccaaaccgggcccctctgctaaccatgttcatgccttcttctttttcctacaggccaccatgaagttatgggatgtcgtggctgtctgcctggtgctgctccacaccgcgtccgccttcccgctgcccgccggtaagaggcctcccgaggcgcccgccgaagaccgctccctcggccgccgccgcgcgcccttcgcgctgagcagtgactcaaatatgccagaggattatcctgatcagttcgatgatgtcatggattttattcaagccaccattaaaagactgaaaaggtcaccagataaacaaatggcagtgcttcctagaagagagcggaatcggcaggctgcagctgccaacccagagaattccagaggaaaaggtcggagaggccagaggggcaaaaaccggggttgtgtcttaactgcaatacatttaaatgtcactgacttgggtctgggctatgaaaccaaggaggaactgatttttaggtactgcagcggctcttgcgatgcagctgagacaacgtacgacaaaatattgaaaaacttatccagaaatagaaggctggtgagtgacaaagtagggcaggcatgttgcagacccatcgcctttgatgatgacctgtcgtttttagatgataacctggtttaccatattctaagaaagcattccgctaaaaggtgtggatgtatctgaaataaagtctgagtgggcggcagcctgtgtgtgcctgggttctctctgtcccggaatgtgcaaacaatggaggtgaagcttcgttacataacttacggtaaatggcccgcctggctgaccgcccaacgacccccgcccattgacgtcaatagtaacgccaatagggactttccattgacgtcaatgggtggagtatttacggtaaactgcccacttggcagtacatcaagtgtatcatatgccaagtacgccccctattgacgtcaatgacggtaaatggcccgcctggcattgtgcccagtacatgaccttatgggactttcctacttggcagtacatctacgtattagtcatcgctattaccatggtcgaggtgagccccacgttctgcttcactctccccatctcccccccctccccacccccaattttgtatttatttattttttaattattttgtgcagcgatgggggcggggggggggggggggcgcgcgccaggcggggcggggcggggcgaggggcggggcggggcgaggcggagaggtgcggcggcagccaatcagagcggcgcgctccgaaagtttccttttatggcgaggcggcggcggcggcggccctataaaaagcgaagcgcgcggcgggcgggagtcgctgcgcgctgccttcgccccgtgccccgctccgccgccgcctcgcgccgcccgccccggctctgactgaccgcgttactcccacaggtgagcgggcgggacggcccttctcctccgggctgtaattagctgagcaagaggtaagggtttaagggatggttggttggtggggtattaatgtttaattacctggagcacctgcctgaaatcactttttttcaggttgggggattcgaacatcggccgccaccatgaacgccagcgagttcaggaggaggggcaaggagatggtggactacgtggccaactacatggagggcatcgagggcaggcaggtgtaccccgacgtggagcccggctacctgaggcccctgatccccgccgccgccccccaggagcccgacaccttcgaggacatcatcaacgacgtggagaagatcatcatgcccggcgtgacccactggcacagcccctacttcttcgcctacttccccaccgccagcagctaccccgccatgctggccgacatgctgtgcggcgccatcggctgcatcggcttcagctgggccgccagccccgcctgcaccgagctggagaccgtgatgatggactggctgggcaagatgctggagctgcccaaggccttcctgaacgagaaggccggcgagggcggcggcgtgatccagggcagcgccagcgaggccaccctggtggccctgctggccgccaggaccaaggtgatccacaggctgcaggccgccagccccgagctgacccaggccgccatcatggagaagctggtggcctacagcagcgaccaggcccacagcagcgtggagagggccggcctgatcggcggcgtgaagctgaaggccatccccagcgacggcaacttcgccatgagggccagcgccctgcaggaggccctggagagggacaaggccgccggcctgatccccttcttcatggtggccaccctgggcaccaccacctgctgcagcttcgacaacctgctggaggtgggccccatctgcaacaaggaggacatctggctgcacgtggacgccgcctacgccggcagcgccttcatctgccccgagttcaggcacctgctgaacggcgtggagttcgccgacagcttcaacttcaacccccacaagtggctgctggtgaacttcgactgcagcgccatgtgggtgaagaagaggaccgacctgaccggcgccttcaggctggaccccacctacctgaagcacagccaccaggacagcggcctgatcaccgactacaggcactggcagatccccctgggcaggaggttcaggagcctgaagatgtggttcgtgttcaggatgtacggcgtgaagggcctgcaggcctacatcaggaagcacgtgcagctgagccacgagttcgagagcctggtgaggcaggaccccaggttcgagatctgcgtggaggtgatcctgggcctggtgtgcttcaggctgaagggcagcaacaaggtgaacgaggccctgctgcagaggatcaacagcgccaagaagatccacctggtgccctgccacctgagggacaagttcgtgctgaggttcgccatctgcagcaggaccgtggagagcgcccacgtgcagagggcctgggagcacatcaaggagctggccgccgacgtgctgagggccgagagggagtgactcgagtaagatacattgatgagtttggacaaaccacaactagaatgcagtgaaaaaaatgctttatttgtgaaatttgtgatgctattgctttatttgtaaccattataagctgcaataaacaagttcggaccgagcggcagatctaggaacccctagtgatggagttggccactccctctctgcgcgctcgctcgctcactgaggccgggcgaccaaaggtcgcccgacgcccgggctttgcccgggcggcctcagtgagcgagcgagcgcgcagctgcctgcagg

SEQ ID NO: 22 - DNA, 4522 bp, synthetic construct
  source 1..4522: mol_type = other DNA; note = HRPDAAV03-E
cctgcaggcagctgcgcgctcgctcgctcactgaggccgcccgggcaaagcccgggcgtcgggcgacctttggtcgcccggcctcagtgagcgagcgagcgcgcagagagggagtggccaactccatcactaggggttcctatcgatatccgttacataacttacggtaaatggcccgcctggctgaccgcccaacgacccccgcccattgacgtcaataatgacgtatgttcccatagtaacgtcaatagggactttccattgacgtcaatgggtggagtatttacggtaaactgcccacttggcagtacatcaagtgtatcatatgccaagtacgccccctattgacgtcaatgacggtaaatggcccgcctggcattatgcccagtacatgaccttatgggactttcctacttggcagtacatctacgtattagtcatcgctattaccatggtgatgcggttttggcagtacatcaatgggcgtggatagcggtttgactcacggggatttccaagtctccaccccattgacgtcaatgggagtttgttttgcaccaaaatcaacgggactttccaaaatgtcgtaacaactccgccccattgacgcaaatgggcggtaggcgtgtacggtgggaggtctatataagcagagctgccaccatgaagttatgggatgtcgtggctgtctgcctggtgctgctccacaccgcgtccgccttcccgctgcccgccggtaagaggcctcccgaggcgcccgccgaagaccgctccctcggccgccgccgcgcgcccttcgcgctgagcagtgactcaaatatgccagaggattatcctgatcagttcgatgatgtcatggattttattcaagccaccattaaaagactgaaaaggtcaccagataaacaaatggcagtgcttcctagaagagagcggaatcggcaggctgcagctgccaacccagagaattccagaggaaaaggtcggagaggccagaggggcaaaaaccggggttgtgtcttaactgcaatacatttaaatgtcactgacttgggtctgggctatgaaaccaaggaggaactgatttttaggtactgcagcggctcttgcgatgcagctgagacaacgtacgacaaaatattgaaaaacttatccagaaatagaaggctggtgagtgacaaagtagggcaggcatgttgcagacccatcgcctttgatgatgacctgtcgtttttagatgataacctggtttaccatattctaagaaagcattccgctaaaaggtgtggatgtatctgaaataaagtctgagtgggcggcagcctgtgtgtgcctgggttctctctgtcccggaatgtgcaaacaatggaggtgaagcttcgttacataacttacggtaaatggcccgcctggctgaccgcccaacgacccccgcccattgacgtcaatagtaacgccaatagggactttccattgacgtcaatgggtggagtatttacggtaaactgcccacttggcagtacatcaagtgtatcatatgccaagtacgccccctattgacgtcaatgacggtaaatggcccgcctggcattgtgcccagtacatgaccttatgggactttcctacttggcagtacatctacgtattagtcatcgctattaccatggtcgaggtgagccccacgttctgcttcactctccccatctcccccccctccccacccccaattttgtatttatttattttttaattattttgtgcagcgatgggggcggggggggggggggggcgcgcgccaggcggggcggggcggggcgaggggcggggcggggcgaggcggagaggtgcggcggcagccaatcagagcggcgcgctccgaaagtttccttttatggcgaggcggcggcggcggcggccctataaaaagcgaagcgcgcggcgggcgggagtcgctgcgcgctgccttcgccccgtgccccgctccgccgccgcctcgcgccgcccgccccggctctgactgaccgcgttactcccacaggtgagcgggcgggacggcccttctcctccgggctgtaattagctgagcaagaggtaagggtttaagggatggttggttggtggggtattaatgtttaattacctggagcacctgcctgaaatcactttttttcaggttgggggattcgaacatcggccgccaccatgaacgccagcgagttcaggaggaggggcaaggagatggtggactacgtggccaactacatggagggcatcgagggcaggcaggtgtaccccgacgtggagcccggctacctgaggcccctgatccccgccgccgccccccaggagcccgacaccttcgaggacatcatcaacgacgtggagaagatcatcatgcccggcgtgacccactggcacagcccctacttcttcgcctacttccccaccgccagcagctaccccgccatgctggccgacatgctgtgcggcgccatcggctgcatcggcttcagctgggccgccagccccgcctgcaccgagctggagaccgtgatgatggactggctgggcaagatgctggagctgcccaaggccttcctgaacgagaaggccggcgagggcggcggcgtgatccagggcagcgccagcgaggccaccctggtggccctgctggccgccaggaccaaggtgatccacaggctgcaggccgccagccccgagctgacccaggccgccatcatggagaagctggtggcctacagcagcgaccaggcccacagcagcgtggagagggccggcctgatcggcggcgtgaagctgaaggccatccccagcgacggcaacttcgccatgagggccagcgccctgcaggaggccctggagagggacaaggccgccggcctgatccccttcttcatggtggccaccctgggcaccaccacctgctgcagcttcgacaacctgctggaggtgggccccatctgcaacaaggaggacatctggctgcacgtggacgccgcctacgccggcagcgccttcatctgccccgagttcaggcacctgctgaacggcgtggagttcgccgacagcttcaacttcaacccccacaagtggctgctggtgaacttcgactgcagcgccatgtgggtgaagaagaggaccgacctgaccggcgccttcaggctggaccccacctacctgaagcacagccaccaggacagcggcctgatcaccgactacaggcactggcagatccccctgggcaggaggttcaggagcctgaagatgtggttcgtgttcaggatgtacggcgtgaagggcctgcaggcctacatcaggaagcacgtgcagctgagccacgagttcgagagcctggtgaggcaggaccccaggttcgagatctgcgtggaggtgatcctgggcctggtgtgcttcaggctgaagggcagcaacaaggtgaacgaggccctgctgcagaggatcaacagcgccaagaagatccacctggtgccctgccacctgagggacaagttcgtgctgaggttcgccatctgcagcaggaccgtggagagcgcccacgtgcagagggcctgggagcacatcaaggagctggccgccgacgtgctgagggccgagagggagtgactcgagaatcaacctctggattacaaaatttgtgaaagattgactggtattcttaactatgttgctccttttacgctatgtggatacgctgctttaatgcctttgtatcatgctattgcttcccgtatggctttcattttctcctccttgtataaatcctggttgctgtctctttatgaggagttgtggcccgttgtcaggcaacgtggcgtggtgtgcactgtgtttgctgacgcaacccccactggttggggcattgccaccacctgtcagctcctttccgggactttcgctttccccctccctattgccacggcggaactcatcgccgcctgccttgcccgctgctggacaggggctcggctgttgggcactgacaattccgtggtgttgtcggggaaatcatcgtcctttccttggctgctcgcctgtgttgccacctggattctgcgcgggacgtccttctgctacgtcccttcggccctcaatccagcggaccttccttcccgcggcctgctgccggctctgcggcctcttccgcgtcttcgccttcgccctcagacgagtcggatctccctttgggccgcctccccgctaagatacattgatgagtttggacaaaccacaactagaatgcagtgaaaaaaatgctttatttgtgaaatttgtgatgctattgctttatttgtaaccattataagctgcaataaacaagttcggaccgagcggcagatctaggaacccctagtgatggagttggccactccctctctgcgcgctcgctcgctcactgaggccgggcgaccaaaggtcgcccgacgcccgggctttgcccgggcggcctcagtgagcgagcgagcgcgcagctgcctgcagg

SEQ ID NO: 23 - DNA, 4614 bp, synthetic construct
  source 1..4614: mol_type = other DNA; note = HRPDAAV03-F
cctgcaggcagctgcgcgctcgctcgctcactgaggccgcccgggcaaagcccgggcgtcgggcgacctttggtcgcccggcctcagtgagcgagcgagcgcgcagagagggagtggccaactccatcactaggggttcctatcgatatccgttacataacttacggtaaatggcccgcctggctgaccgcccaacgacccccgcccattgacgtcaataatgacgtatgttcccatagtaacgtcaatagggactttccattgacgtcaatgggtggagtatttacggtaaactgcccacttggcagtacatcaagtgtatcatatgccaagtacgccccctattgacgtcaatgacggtaaatggcccgcctggcattatgcccagtacatgaccttatgggactttcctacttggcagtacatctacgtattagtcatcgctattaccatggtgatgcggttttggcagtacatcaatgggcgtggatagcggtttgactcacggggatttccaagtctccaccccattgacgtcaatgggagtttgttttgcaccaaaatcaacgggactttccaaaatgtcgtaacaactccgccccattgacgcaaatgggcggtaggcgtgtacggtgggaggtctatataagcagagctaagaggtaagggtttaagggatggttggttggtggggtattaatgtttaattacctggagcacctgcctgaaatcactttttttcaggttgggccaccatgaagttatgggatgtcgtggctgtctgcctggtgctgctccacaccgcgtccgccttcccgctgcccgccggtaagaggcctcccgaggcgcccgccgaagaccgctccctcggccgccgccgcgcgcccttcgcgctgagcagtgactcaaatatgccagaggattatcctgatcagttcgatgatgtcatggattttattcaagccaccattaaaagactgaaaaggtcaccagataaacaaatggcagtgcttcctagaagagagcggaatcggcaggctgcagctgccaacccagagaattccagaggaaaaggtcggagaggccagaggggcaaaaaccggggttgtgtcttaactgcaatacatttaaatgtcactgacttgggtctgggctatgaaaccaaggaggaactgatttttaggtactgcagcggctcttgcgatgcagctgagacaacgtacgacaaaatattgaaaaacttatccagaaatagaaggctggtgagtgacaaagtagggcaggcatgttgcagacccatcgcctttgatgatgacctgtcgtttttagatgataacctggtttaccatattctaagaaagcattccgctaaaaggtgtggatgtatctgaaataaagtctgagtgggcggcagcctgtgtgtgcctgggttctctctgtcccggaatgtgcaaacaatggaggtgaagcttcgttacataacttacggtaaatggcccgcctggctgaccgcccaacgacccccgcccattgacgtcaatagtaacgccaatagggactttccattgacgtcaatgggtggagtatttacggtaaactgcccacttggcagtacatcaagtgtatcatatgccaagtacgccccctattgacgtcaatgacggtaaatggcccgcctggcattgtgcccagtacatgaccttatgggactttcctacttggcagtacatctacgtattagtcatcgctattaccatggtcgaggtgagccccacgttctgcttcactctccccatctcccccccctccccacccccaattttgtatttatttattttttaattattttgtgcagcgatgggggcggggggggggggggggcgcgcgccaggcggggcggggcggggcgaggggcggggcggggcgaggcggagaggtgcggcggcagccaatcagagcggcgcgctccgaaagtttccttttatggcgaggcggcggcggcggcggccctataaaaagcgaagcgcgcggcgggcgggagtcgctgcgcgctgccttcgccccgtgccccgctccgccgccgcctcgcgccgcccgccccggctctgactgaccgcgttactcccacaggtgagcgggcgggacggcccttctcctccgggctgtaattagctgagcaagaggtaagggtttaagggatggttggttggtggggtattaatgtttaattacctggagcacctgcctgaaatcactttttttcaggttgggggattcgaacatcggccgccaccatgaacgccagcgagttcaggaggaggggcaaggagatggtggactacgtggccaactacatggagggcatcgagggcaggcaggtgtaccccgacgtggagcccggctacctgaggcccctgatccccgccgccgccccccaggagcccgacaccttcgaggacatcatcaacgacgtggagaagatcatcatgcccggcgtgacccactggcacagcccctacttcttcgcctacttccccaccgccagcagctaccccgccatgctggccgacatgctgtgcggcgccatcggctgcatcggcttcagctgggccgccagccccgcctgcaccgagctggagaccgtgatgatggactggctgggcaagatgctggagctgcccaaggccttcctgaacgagaaggccggcgagggcggcggcgtgatccagggcagcgccagcgaggccaccctggtggccctgctggccgccaggaccaaggtgatccacaggctgcaggccgccagccccgagctgacccaggccgccatcatggagaagctggtggcctacagcagcgaccaggcccacagcagcgtggagagggccggcctgatcggcggcgtgaagctgaaggccatccccagcgacggcaacttcgccatgagggccagcgccctgcaggaggccctggagagggacaaggccgccggcctgatccccttcttcatggtggccaccctgggcaccaccacctgctgcagcttcgacaacctgctggaggtgggccccatctgcaacaaggaggacatctggctgcacgtggacgccgcctacgccggcagcgccttcatctgccccgagttcaggcacctgctgaacggcgtggagttcgccgacagcttcaacttcaacccccacaagtggctgctggtgaacttcgactgcagcgccatgtgggtgaagaagaggaccgacctgaccggcgccttcaggctggaccccacctacctgaagcacagccaccaggacagcggcctgatcaccgactacaggcactggcagatccccctgggcaggaggttcaggagcctgaagatgtggttcgtgttcaggatgtacggcgtgaagggcctgcaggcctacatcaggaagcacgtgcagctgagccacgagttcgagagcctggtgaggcaggaccccaggttcgagatctgcgtggaggtgatcctgggcctggtgtgcttcaggctgaagggcagcaacaaggtgaacgaggccctgctgcagaggatcaacagcgccaagaagatccacctggtgccctgccacctgagggacaagttcgtgctgaggttcgccatctgcagcaggaccgtggagagcgcccacgtgcagagggcctgggagcacatcaaggagctggccgccgacgtgctgagggccgagagggagtgactcgagaatcaacctctggattacaaaatttgtgaaagattgactggtattcttaactatgttgctccttttacgctatgtggatacgctgctttaatgcctttgtatcatgctattgcttcccgtatggctttcattttctcctccttgtataaatcctggttgctgtctctttatgaggagttgtggcccgttgtcaggcaacgtggcgtggtgtgcactgtgtttgctgacgcaacccccactggttggggcattgccaccacctgtcagctcctttccgggactttcgctttccccctccctattgccacggcggaactcatcgccgcctgccttgcccgctgctggacaggggctcggctgttgggcactgacaattccgtggtgttgtcggggaaatcatcgtcctttccttggctgctcgcctgtgttgccacctggattctgcgcgggacgtccttctgctacgtcccttcggccctcaatccagcggaccttccttcccgcggcctgctgccggctctgcggcctcttccgcgtcttcgccttcgccctcagacgagtcggatctccctttgggccgcctccccgctaagatacattgatgagtttggacaaaccacaactagaatgcagtgaaaaaaatgctttatttgtgaaatttgtgatgctattgctttatttgtaaccattataagctgcaataaacaagttcggaccgagcggcagatctaggaacccctagtgatggagttggccactccctctctgcgcgctcgctcgctcactgaggccgggcgaccaaaggtcgcccgacgcccgggctttgcccgggcggcctcagtgagcgagcgagcgcgcagctgcctgcagg

SEQ ID NO: 24 - DNA, 3988 bp, synthetic construct
  source 1..3988: mol_type = other DNA; note = HRPDAAV02-AI
cctgcaggcagctgcgcgctcgctcgctcactgaggccgcccgggcaaagcccgggcgtcgggcgacctttggtcgcccggcctcagtgagcgagcgagcgcgcagagagggagtggccaactccatcactaggggttcctatcgatatcaagcttcgttacataacttacggtaaatggcccgcctggctgaccgcccaacgacccccgcccattgacgtcaatagtaacgccaatagggactttccattgacgtcaatgggtggagtatttacggtaaactgcccacttggcagtacatcaagtgtatcatatgccaagtacgccccctattgacgtcaatgacggtaaatggcccgcctggcattgtgcccagtacatgaccttatgggactttcctacttggcagtacatctacgtattagtcatcgctattaccatggtcgaggtgagccccacgttctgcttcactctccccatctcccccccctccccacccccaattttgtatttatttattttttaattattttgtgcagcgatgggggcggggggggggggggggcgcgcgccaggcggggcggggcggggcgaggggcggggcggggcgaggcggagaggtgcggcggcagccaatcagagcggcgcgctccgaaagtttccttttatggcgaggcggcggcggcggcggccctataaaaagcgaagcgcgcggcgggcgggagtcgctgcgcgctgccttcgccccgtgccccgctccgccgccgcctcgcgccgcccgccccggctctgactgaccgcgttactcccacaggtgagcgggcgggacggcccttctcctccgggctgtaattagctgagcaagaggtaagggtttaagggatggttggttggtggggtattaatgtttaattacctggagcacctgcctgaaatcactttttttcaggttgggggattcgaacatcggccgccaccatgaatgctagcgagtttcgcagaaggggcaaggagatggtggattacgtggctaattacatggagggcatcgagggccggcaggtgtacccagatgtggagccaggctacctgagaccactgatccctgctgccgccccacaggagccagacaccttcgaggatatcatcaatgacgtggagaagatcatcatgcctggcgtgacccactggcatagcccatacttctttgcctactttccaacagcctcttcctatcccgctatgctggctgatatgctgtgcggcgctatcggctgcatcggcttctcttgggccgctagccctgcttgcacagagctggagaccgtgatgatggattggctgggcaagatgctggagctgcctaaggcctttctgaacgagaaggctggcgagggcggcggcgtgatccagggctctgcctccgaggctacactggtggctctgctggctgcccggacaaaggtaatccacagactgcaggctgcctctccagagctgacccaggccgctatcatggagaagctggtggcttactctagcgaccaggctcattcttccgtggagcgggctggcctgatcggcggcgtgaagctgaaggccatcccttccgacggcaatttcgccatgagagcttctgccctgcaggaggctctggagagagataaggctgccggcctgatccctttctttatggtggccaccctgggcacaaccacctgttgctccttcgacaacctgctggaggtgggccctatctgtaacaaggaggacatctggctgcatgtggatgccgcttatgctggctctgcctttatctgccccgagtttagacatctgctgaacggcgtggagtttgccgacagctttaacttcaaccctcacaagtggctgctggtgaattttgactgctctgccatgtgggtgaagaagaggacagacctgaccggcgcttttaggctggatccaacctacctgaagcacagccatcaggacagcggcctgatcacagactacagacactggcagatcccactgggcagaaggtttcggtctctgaagatgtggttcgtgtttcgcatgtatggcgtgaagggcctgcaggcttatatccggaagcacgtgcagctgtctcatgagttcgagtccctggtgcggcaggacccaagatttgagatctgcgtggaggtaatcctgggcctggtgtgcttcaggctgaagggctctaataaggtgaacgaggctctgctgcagaggatcaacagcgccaagaagatccatctggtgccttgtcatctgagggacaagttcgtgctgagattcgccatctgctctagaacagtggagtctgctcatgtgcagagggcttgggagcatatcaaggagctggccgctgacgtgctgagggctgagagggaggccaccaacttctccctgctgaagcaggccggcgacgtggaggagaaccccggccccatgaagctgtgggatgtggtggccgtgtgcctggtgctgctgcacaccgcttctgccttcccactgcctgccggcaagagacctcccgaggcccctgccgaggacagaagcctgggcaggcggagagccccatttgctctgtctagcgattccaacatgcctgaggattaccccgatcagttcgatgacgtgatggatttcatccaggccaccatcaagagactgaagagatctcctgacaagcagatggctgtgctgcctagaagggagagaaacaggcaggccgctgctgccaatccagagaactccaggggcaagggcagaaggggccagcgcggcaagaatagaggctgcgtgctgacagccatccacctgaacgtgaccgacctgggcctgggctacgagaccaaggaggagctgatcttcaggtactgtagcggctcctgtgatgctgccgagaccacatacgacaagatcctgaagaacctgtccaggaacagaaggctggtgtctgacaaggtgggccaggcttgctgtaggccaatcgctttcgacgacgatctgtcctttctggatgacaacctggtgtaccacatcctgaggaagcattccgctaagagatgtggctgcatctgactcgagaatcaacctctggattacaaaatttgtgaaagattgactggtattcttaactatgttgctccttttacgctatgtggatacgctgctttaatgcctttgtatcatgctattgcttcccgtatggctttcattttctcctccttgtataaatcctggttgctgtctctttatgaggagttgtggcccgttgtcaggcaacgtggcgtggtgtgcactgtgtttgctgacgcaacccccactggttggggcattgccaccacctgtcagctcctttccgggactttcgctttccccctccctattgccacggcggaactcatcgccgcctgccttgcccgctgctggacaggggctcggctgttgggcactgacaattccgtggtgttgtcggggaaatcatcgtcctttccttggctgctcgcctgtgttgccacctggattctgcgcgggacgtccttctgctacgtcccttcggccctcaatccagcggaccttccttcccgcggcctgctgccggctctgcggcctcttccgcgtcttcgccttcgccctcagacgagtcggatctccctttgggccgcctccccgctaagatacattgatgagtttggacaaaccacaactagaatgcagtgaaaaaaatgctttatttgtgaaatttgtgatgctattgctttatttgtaaccattataagctgcaataaacaagttcggaccgagcggcagatctaggaacccctagtgatggagttggccactccctctctgcgcgctcgctcgctcactgaggccgggcgaccaaaggtcgcccgacgcccgggctttgcccgggcggcctcagtgagcgagcgagcgcgcagctgcctgcagg

SEQ ID NO: 25 - DNA, 4503 bp, synthetic construct
  source 1..4503: mol_type = other DNA; note = HRPDAAV03-DI
cctgcaggcagctgcgcgctcgctcgctcactgaggccgcccgggcaaagcccgggcgtcgggcgacctttggtcgcccggcctcagtgagcgagcgagcgcgcagagagggagtggccaactccatcactaggggttcctatcgatatccgttacataacttacggtaaatggcccgcctggctgaccgcccaacgacccccgcccattgacgtcaataatgacgtatgttcccatagtaacgtcaatagggactttccattgacgtcaatgggtggagtatttacggtaaactgcccacttggcagtacatcaagtgtatcatatgccaagtacgccccctattgacgtcaatgacggtaaatggcccgcctggcattatgcccagtacatgaccttatgggactttcctacttggcagtacatctacgtattagtcatcgctattaccatggtgatgcggttttggcagtacatcaatgggcgtggatagcggtttgactcacggggatttccaagtctccaccccattgacgtcaatgggagtttgttttgcaccaaaatcaacgggactttccaaaatgtcgtaacaactccgccccattgacgcaaatgggcggtaggcgtgtacggtgggaggtctatataagcagagctgtgagtttggggacccttgattgttctttctttttcgctattgtaaaattcatgttatatggagggggcaaagttttcagggtgttgtttagaatgggaagatgtcccttgtatcaccatggaccctcatgataattttgtttctttcactttctactctgttgacaaccattgtctcctcttattttcttttcattttctgtaactttttcgttaaactttagcttgcatttgtaacgaatttttaaattcacttttgtttatttgtcagattgtaagtactttctctaatcacttttttttcaaggcaatcagggtatattatattgtacttcagcacagttttagagaacaattgttataattaaatgataaggtagaatatttctgcatataaattctggctggcgtggaaatattcttattggtagaaacaactacatcctggtcatcatcctgcctttctctttatggttacaatgatatacactgtttgagatgaggataaaatactctgagtccaaaccgggcccctctgctaaccatgttcatgccttcttctttttcctacaggccaccatgaagctgtgggatgtggtggccgtgtgcctggtgctgctgcacaccgcttctgccttcccactgcctgccggcaagagacctcccgaggcccctgccgaggacagaagcctgggcaggcggagagccccatttgctctgtctagcgattccaacatgcctgaggattaccccgatcagttcgatgacgtgatggatttcatccaggccaccatcaagagactgaagagatctcctgacaagcagatggctgtgctgcctagaagggagagaaacaggcaggccgctgctgccaatccagagaactccaggggcaagggcagaaggggccagcgcggcaagaatagaggctgcgtgctgacagccatccacctgaacgtgaccgacctgggcctgggctacgagaccaaggaggagctgatcttcaggtactgtagcggctcctgtgatgctgccgagaccacatacgacaagatcctgaagaacctgtccaggaacagaaggctggtgtctgacaaggtgggccaggcttgctgtaggccaatcgctttcgacgacgatctgtcctttctggatgacaacctggtgtaccacatcctgaggaagcattccgctaagagatgtggctgcatctgaaataaagtctgagtgggcggcagcctgtgtgtgcctgggttctctctgtcccggaatgtgcaaacaatggaggtgaagcttcgttacataacttacggtaaatggcccgcctggctgaccgcccaacgacccccgcccattgacgtcaatagtaacgccaatagggactttccattgacgtcaatgggtggagtatttacggtaaactgcccacttggcagtacatcaagtgtatcatatgccaagtacgccccctattgacgtcaatgacggtaaatggcccgcctggcattgtgcccagtacatgaccttatgggactttcctacttggcagtacatctacgtattagtcatcgctattaccatggtcgaggtgagccccacgttctgcttcactctccccatctcccccccctccccacccccaattttgtatttatttattttttaattattttgtgcagcgatgggggcggggggggggggggggcgcgcgccaggcggggcggggcggggcgaggggcggggcggggcgaggcggagaggtgcggcggcagccaatcagagcggcgcgctccgaaagtttccttttatggcgaggcggcggcggcggcggccctataaaaagcgaagcgcgcggcgggcgggagtcgctgcgcgctgccttcgccccgtgccccgctccgccgccgcctcgcgccgcccgccccggctctgactgaccgcgttactcccacaggtgagcgggcgggacggcccttctcctccgggctgtaattagctgagcaagaggtaagggtttaagggatggttggttggtggggtattaatgtttaattacctggagcacctgcctgaaatcactttttttcaggttgggggattcgaacatcggccgccaccatgaatgctagcgagtttcgcagaaggggcaaggagatggtggattacgtggctaattacatggagggcatcgagggccggcaggtgtacccagatgtggagccaggctacctgagaccactgatccctgctgccgccccacaggagccagacaccttcgaggatatcatcaatgacgtggagaagatcatcatgcctggcgtgacccactggcatagcccatacttctttgcctactttccaacagcctcttcctatcccgctatgctggctgatatgctgtgcggcgctatcggctgcatcggcttctcttgggccgctagccctgcttgcacagagctggagaccgtgatgatggattggctgggcaagatgctggagctgcctaaggcctttctgaacgagaaggctggcgagggcggcggcgtgatccagggctctgcctccgaggctacactggtggctctgctggctgcccggacaaaggtaatccacagactgcaggctgcctctccagagctgacccaggccgctatcatggagaagctggtggcttactctagcgaccaggctcattcttccgtggagcgggctggcctgatcggcggcgtgaagctgaaggccatcccttccgacggcaatttcgccatgagagcttctgccctgcaggaggctctggagagagataaggctgccggcctgatccctttctttatggtggccaccctgggcacaaccacctgttgctccttcgacaacctgctggaggtgggccctatctgtaacaaggaggacatctggctgcatgtggatgccgcttatgctggctctgcctttatctgccccgagtttagacatctgctgaacggcgtggagtttgccgacagctttaacttcaaccctcacaagtggctgctggtgaattttgactgctctgccatgtgggtgaagaagaggacagacctgaccggcgcttttaggctggatccaacctacctgaagcacagccatcaggacagcggcctgatcacagactacagacactggcagatcccactgggcagaaggtttcggtctctgaagatgtggttcgtgtttcgcatgtatggcgtgaagggcctgcaggcttatatccggaagcacgtgcagctgtctcatgagttcgagtccctggtgcggcaggacccaagatttgagatctgcgtggaggtaatcctgggcctggtgtgcttcaggctgaagggctctaataaggtgaacgaggctctgctgcagaggatcaacagcgccaagaagatccatctggtgccttgtcatctgagggacaagttcgtgctgagattcgccatctgctctagaacagtggagtctgctcatgtgcagagggcttgggagcatatcaaggagctggccgctgacgtgctgagggctgagagggagctcgagtaagatacattgatgagtttggacaaaccacaactagaatgcagtgaaaaaaatgctttatttgtgaaatttgtgatgctattgctttatttgtaaccattataagctgcaataaacaagttcggaccgagcggcagatctaggaacccctagtgatggagttggccactccctctctgcgcgctcgctcgctcactgaggccgggcgaccaaaggtcgcccgacgcccgggctttgcccgggcggcctcagtgagcgagcgagcgcgcagctgcctgcagg

SEQ ID NO: 26 - DNA, 141 bp, synthetic construct
  source 1..141: mol_type = other DNA; note = 5 ITR
cctgcaggcagctgcgcgctcgctcgctcactgaggccgcccgggcaaagcccgggcgtcgggcgacctttggtcgcccggcctcagtgagcgagcgagcgcgcagagagggagtggccaactccatcactaggggttcct

SEQ ID NO: 27 - DNA, 286 bp, synthetic construct
  source 1..286: mol_type = other DNA; note = CMV enhancer 1
cgttacataacttacggtaaatggcccgcctggctgaccgcccaacgacccccgcccattgacgtcaatagtaacgccaatagggactttccattgacgtcaatgggtggagtatttacggtaaactgcccacttggcagtacatcaagtgtatcatatgccaagtacgccccctattgacgtcaatgacggtaaatggcccgcctggcattgtgcccagtacatgaccttatgggactttcctacttggcagtacatctacgtattagtcatcgctattaccatg

SEQ ID NO: 28 - DNA, 278 bp, synthetic construct
  source 1..278: mol_type = other DNA; note = CBA promoter
tcgaggtgagccccacgttctgcttcactctccccatctcccccccctccccacccccaattttgtatttatttattttttaattattttgtgcagcgatgggggcggggggggggggggggcgcgcgccaggcggggcggggcggggcgaggggcggggcggggcgaggcggagaggtgcggcggcagccaatcagagcggcgcgctccgaaagtttccttttatggcgaggcggcggcggcggcggccctataaaaagcgaagcgcgcggcgggcg

SEQ ID NO: 29 - DNA, 228 bp, synthetic construct
  source 1..228: mol_type = other DNA; note = hybrid intron
ggagtcgctgcgcgctgccttcgccccgtgccccgctccgccgccgcctcgcgccgcccgccccggctctgactgaccgcgttactcccacaggtgagcgggcgggacggcccttctcctccgggctgtaattagctgagcaagaggtaagggtttaagggatggttggttggtggggtattaatgtttaattacctggagcacctgcctgaaatcactttttttcag

SEQ ID NO: 30 - DNA, 477 bp, synthetic construct
  source 1..477: mol_type = other DNA; note = hGH poly(A)
gggtggcatccctgtgacccctccccagtgcctctcctggccctggaagttgccactccagtgcccaccagccttgtcctaataaaattaagttgcatcattttgtctgactaggtgtccttctataatattatggggtggaggggggtggtatggagcaaggggcaagttgggaagacaacctgtagggcctgcggggtctattgggaaccaagctggagtgcagtggcacaatcttggctcactgcaatctccgcctcctgggttcaagcgattctcctgcctcagcctcccgagttgttgggattccaggcatgcatgaccaggctcagctaatttttgtttttttggtagagacggggtttcaccatattggccaggctggtctccaactcctaatctcaggtgatctacccaccttggcctcccaaattgctgggattacaggcgtgaaccactgctcccttccctgtcctt

SEQ ID NO: 31 - DNA, 141 bp, synthetic construct
  source 1..141: mol_type = other DNA; note = 3 ITR
aggaacccctagtgatggagttggccactccctctctgcgcgctcgctcgctcactgaggccgggcgaccaaaggtcgcccgacgcccgggctttgcccgggcggcctcagtgagcgagcgagcgcgcagctgcctgcagg

SEQ ID NO: 32 - DNA, 122 bp, synthetic construct
  source 1..122: mol_type = other DNA; note = SV40 poly(A)
taagatacattgatgagtttggacaaaccacaactagaatgcagtgaaaaaaatgctttatttgtgaaatttgtgatgctattgctttatttgtaaccattataagctgcaataaacaagtt

SEQ ID NO: 33 - DNA, 726 bp, synthetic construct
  source 1..726: mol_type = other DNA; note = HPRE
ataacaggcctattgattggaaagtttgtcaacgaattgtgggtcttttggggtttgctgccccttttacgcaatgtggatatcctgctttaatgcctttatatgcatgtatacaagcaaaacaggcttttactttctcgccaacttacaaggcctttctcagtaaacagtatatgaccctttaccccgttgctcggcaacggcctggtctgtgccaagtgtttgctgacgcaacccccactggttggggcttggccataggccatcagcgcatgcgtggaacctttgtgtctcctctgccgatccatactgcggaactcctagccgcttgttttgctcgcagcaggtctggagcaaacctcatcgggaccgacaattctgtcgtactctcccgcaagtatacatcgtttccatggctgctaggctgtgctgccaactggatcctgcgcgggacgtcctttgtttacgtcccgtcggcgctgaatcccgcggacgacccctcccggggccgcttggggctctaccgcccgcttctccgtctgccgtaccgtccgaccacggggcgcacctctctttacgcggactccccgtctgtgccttctcatctgccggaccgtgtgcacttcgcttcacctctgcacgtcgcatggaggccaccgtgaacgcccaccggaacctgcccaaggtcttgcataagaggactcttggactttcagcaatgtcatc

SEQ ID NO: 34 - DNA, 589 bp, synthetic construct
  source 1..589: mol_type = other DNA; note = WPRE
aatcaacctctggattacaaaatttgtgaaagattgactggtattcttaactatgttgctccttttacgctatgtggatacgctgctttaatgcctttgtatcatgctattgcttcccgtatggctttcattttctcctccttgtataaatcctggttgctgtctctttatgaggagttgtggcccgttgtcaggcaacgtggcgtggtgtgcactgtgtttgctgacgcaacccccactggttggggcattgccaccacctgtcagctcctttccgggactttcgctttccccctccctattgccacggcggaactcatcgccgcctgccttgcccgctgctggacaggggctcggctgttgggcactgacaattccgtggtgttgtcggggaaatcatcgtcctttccttggctgctcgcctgtgttgccacctggattctgcgcgggacgtccttctgctacgtcccttcggccctcaatccagcggaccttccttcccgcggcctgctgccggctctgcggcctcttccgcgtcttcgccttcgccctcagacgagtcggatctccctttgggccgcctccccgc

SEQ ID NO: 35 - DNA, 203 bp, synthetic construct
  source 1..203: mol_type = other DNA; note = CMV promoter
gtgatgcggttttggcagtacatcaatgggcgtggatagcggtttgactcacggggatttccaagtctccaccccattgacgtcaatgggagtttgttttgcaccaaaatcaacgggactttccaaaatgtcgtaacaactccgccccattgacgcaaatgggcggtaggcgtgtacggtgggaggtctatataagcagagct

SEQ ID NO: 36 - DNA, 1268 bp, synthetic construct
  source 1..1268: mol_type = other DNA; note = PA75 polyA
aataaagtctgagtgggcggcagcctgtgtgtgcctgggttctctctgtcccggaatgtgcaaacaatggaggtgggcctacatcaggaagcacgtgcagctgagccacgagttcgagagcctggtgaggcaggaccccaggttcgagatctgcgtggaggtgatcctgggcctggtgtgcttcaggctgaagggcagcaacaaggtgaacgaggccctgctgcagaggatcaacagcgccaagaagatccacctggtgccctgccacctgagggacaagttcgtgctgaggttcgccatctgcagcaggaccgtggagagcgcccacgtgcagagggcctgggagcacatcaaggagctggccgccgacgtgctgagggccgagagggagtgactcgagtaagatacattgatgagtttggacaaaccacaactagaatgcagtgaaaaaaatgctttatttgtgaaatttgtgatgctattgctttatttgtaaccattataagctgcaataaacaagttcgttacataacttacggtaaatggcccgcctggctgaccgcccaacgacccccgcccattgacgtcaataatgacgtatgttcccatagtaacgtcaatagggactttccattgacgtcaatgggtggagtatttacggtaaactgcccacttggcagtacatcaagtgtatcatatgccaagtacgccccctattgacgtcaatgacggtaaatggcccgcctggcattatgcccagtacatgaccttatgggactttcctacttggcagtacatctacgtattagtcatcgctattaccatggtgatgcggttttggcagtacatcaatgggcgtggatagcggtttgactcacggggatttccaagtctccaccccattgacgtcaatgggagtttgttttgcaccaaaatcaacgggactttccaaaatgtcgtaacaactccgccccattgacgcaaatgggcggtaggcgtgtacggtgggaggtctatataagcagagctgccaccatgaagttatgggatgtcgtggctgtctgcctggtgctgctccacaccgcgtccgccttcccgctgcccgccggtaagaggcctcccgaggcgcccgccgaagaccgctccctcggccgccgccgcgcgcccttcgcgctgagcagtgactcaaatatgccagaggattatcctgatcagttcgatgatgtcatggattttattcaagccaccattaaaagactgaaaaggtc

SEQ ID NO: 37 - DNA, 304 bp, synthetic construct
  source 1..304: mol_type = other DNA; note = CMV Enhancer2
cgttacataacttacggtaaatggcccgcctggctgaccgcccaacgacccccgcccattgacgtcaataatgacgtatgttcccatagtaacgtcaatagggactttccattgacgtcaatgggtggagtatttacggtaaactgcccacttggcagtacatcaagtgtatcatatgccaagtacgccccctattgacgtcaatgacggtaaatggcccgcctggcattatgcccagtacatgaccttatgggactttcctacttggcagtacatctacgtattagtcatcgctattaccatg

SEQ ID NO: 38 - DNA, 573 bp, synthetic construct
  source 1..573: mol_type = other DNA; note = globin intron
gtgagtttggggacccttgattgttctttctttttcgctattgtaaaattcatgttatatggagggggcaaagttttcagggtgttgtttagaatgggaagatgtcccttgtatcaccatggaccctcatgataattttgtttctttcactttctactctgttgacaaccattgtctcctcttattttcttttcattttctgtaactttttcgttaaactttagcttgcatttgtaacgaatttttaaattcacttttgtttatttgtcagattgtaagtactttctctaatcacttttttttcaaggcaatcagggtatattatattgtacttcagcacagttttagagaacaattgttataattaaatgataaggtagaatatttctgcatataaattctggctggcgtggaaatattcttattggtagaaacaactacatcctggtcatcatcctgcctttctctttatggttacaatgatatacactgtttgagatgaggataaaatactctgagtccaaaccgggcccctctgctaaccatgttcatgccttcttctttttcctacag

SEQ ID NO: 39 - DNA, 92 bp, synthetic construct
  source 1..92: mol_type = other DNA; note = MVM intron
aagaggtaagggtttaagggatggttggttggtggggtattaatgtttaattacctggagcacctgcctgaaatcactttttttcaggttgg

SEQ ID NO: 40 - DNA, 16 bp, synthetic construct
  source 1..16: mol_type = other DNA; note = MCS
atcgatatccgttaca

SEQ ID NO: 41 - DNA, 2208 bp, synthetic construct
  source 1..2208: mol_type = other DNA; note = AAV2
atggctgccgatggttatcttccagattggctcgaggacactctctctgaaggaataagacagtggtggaagctcaaacctggcccaccaccaccaaagcccgcagagcggcataaggacgacagcaggggtcttgtgcttcctgggtacaagtacctcggacccttcaacggactcgacaagggagagccggtcaacgaggcagacgccgcggccctcgagcacgacaaagcctacgaccggcagctcgacagcggagacaacccgtacctcaagtacaaccacgccgacgcggagtttcaggagcgccttaaagaagatacgtcttttgggggcaacctcggacgagcagtcttccaggcgaaaaagagggttcttgaacctctgggcctggttgaggaacctgttaagacggctccgggaaaaaagaggccggtagagcactctcctgtggagccagactcctcctcgggaaccggaaaggcgggccagcagcctgcaagaaaaagattgaattttggtcagactggagacgcagactcagtacctgacccccagcctctcggacagccaccagcagccccctctggtctgggaactaatacgatggctacaggcagtggcgcaccaatggcagacaataacgagggcgccgacggagtgggtaattcctcgggaaattggcattgcgattccacatggatgggcgacagagtcatcaccaccagcacccgaacctgggccctgcccacctacaacaaccacctctacaaacaaatttccagccaatcaggagcctcgaacgacaatcactactttggctacagcaccccttgggggtattttgacttcaacagattccactgccacttttcaccacgtgactggcaaagactcatcaacaacaactggggattccgacccaagagactcaacttcaagctctttaacattcaagtcaaagaggtcacgcagaatgacggtacgacgacgattgccaataaccttaccagcacggttcaggtgtttactgactcggagtaccagctcccgtacgtcctcggctcggcgcatcaaggatgcctcccgccgttcccagcagacgtcttcatggtgccacagtatggatacctcaccctgaacaacgggagtcaggcagtaggacgctcttcattttactgcctggagtactttccttctcagatgctgcgtaccggaaacaactttaccttcagctacacttttgaggacgttcctttccacagcagctacgctcacagccagagtctggaccgtctcatgaatcctctcatcgaccagtacctgtattacttgagcagaacaaacactccaagtggaaccaccacgcagtcaaggcttcagttttctcaggccggagcgagtgacattcgggaccagtctaggaactggcttcctggaccctgttaccgccagcagcgagtatcaaagacatctgcggataacaacaacagtgaatactcgtggactggagctaccaagtaccacctcaatggcagagactctctggtgaatccgggcccggccatggcaagccacaaggacgatgaagaaaagttttttcctcagagcggggttctcatctttgggaagcaaggctcagagaaaacaaatgtggacattgaaaaggtcatgattacagacgaagaggaaatcaggacaaccaatcccgtggctacggagcagtatggttctgtatctaccaacctccagagaggcaacagacaagcagctaccgcagatgtcaacacacaaggcgttcttccaggcatggtctggcaggacagagatgtgtaccttcaggggcccatctgggcaaagattccacacacggacggacattttcacccctctcccctcatgggtggattcggacttaaacaccctcctccacagattctcatcaagaacaccccggtacctgcgaatccttcgaccaccttcagtgcggcaaagtttgcttccttcatcacacagtactccacgggacaggtcagcgtggagatcgagtgggagctgcagaaggaaaacagcaaacgctggaatcccgaaattcagtacacttccaactacaacaagtctgttaatgtggactttactgtggacactaatggcgtgtattcagagcctcgccccattggcaccagatacctgactcgtaatctgtaa

SEQ ID NO: 42 - DNA, 2211 bp, synthetic construct
  source 1..2211: mol_type = other DNA; note = AAV9
atggctgccgatggttatcttccagattggctcgaggacaaccttagtgaaggaattcgcgagtggtgggctttgaaacctggagcccctcaacccaaggcaaatcaacaacatcaagacaacgctcgaggtcttgtgcttccgggttacaaataccttggacccggcaacggactcgacaagggggagccggtcaacgcagcagacgcggcggccctcgagcacgacaaggcctacgaccagcagctcaaggccggagacaacccgtacctcaagtacaaccacgccgacgccgagttccaggagcggctcaaagaagatacgtcttttgggggcaacctcgggcgagcagtcttccaggccaaaaagaggcttcttgaacctcttggtctggttgaggaagcggctaagacggctcctggaaagaagaggcctgtagagcagtctcctcaggaaccggactcctccgcgggtattggcaaatcgggtgcacagcccgctaaaaagagactcaatttcggtcagactggcgacacagagtcagtcccagaccctcaaccaatcggagaacctcccgcagccccctcaggtgtgggatctcttacaatggcttcaggtggtggcgcaccagtggcagacaataacgaaggtgccgatggagtgggtagttcctcgggaaattggcattgcgattcccaatggctgggggacagagtcatcaccaccagcacccgaacctgggccctgcccacctacaacaatcacctctacaagcaaatctccaacagcacatctggaggatcttcaaatgacaacgcctacttcggctacagcaccccctgggggtattttgacttcaacagattccactgccacttctcaccacgtgactggcagcgactcatcaacaacaactggggattccggcctaagcgactcaacttcaagctcttcaacattcaggtcaaagaggttacggacaacaatggagtcaagaccatcgccaataaccttaccagcacggtccaggtcttcacggactcagactatcagctcccgtacgtgctcgggtcggctcacgagggctgcctcccgccgttcccagcggacgttttcatgattcctcagtacgggtatctgacgcttaatgatggaagccaggccgtgggtcgttcgtccttttactgcctggaatatttcccgtcgcaaatgctaagaacgggtaacaacttccagttcagctacgagtttgagaacgtacctttccatagcagctacgctcacagccaaagcctggaccgactaatgaatccactcatcgaccaatacttgtactatctctcaaagactattaacggttctggacagaatcaacaaacgctaaaattcagtgtggccggacccagcaacatggctgtccagggaagaaactacatacctggacccagctaccgacaacaacgtgtctcaaccactgtgactcaaaacaacaacagcgaatttgcttggcctggagcttcttcttgggctctcaatggacgtaatagcttgatgaatcctggacctgctatggccagccacaaagaaggagaggaccgtttctttcctttgtctggatctttaatttttggcaaacaaggaactggaagagacaacgtggatgcggacaaagtcatgataaccaacgaagaagaaattaaaactactaacccggtagcaacggagtcctatggacaagtggccacaaaccaccagagtgcccaagcacaggcgcagaccggctgggttcaaaaccaaggaatacttccgggtatggtttggcaggacagagatgtgtacctgcaaggacccatttgggccaaaattcctcacacggacggcaactttcacccttctccgctgatgggagggtttggaatgaagcacccgcctcctcagatcctcatcaaaaacacacctgtacctgcggatcctccaacggccttcaacaaggacaagctgaactctttcatcacccagtattctactggccaagtcagcgtggagatcgagtgggagctgcagaaggaaaacagcaagcgctggaacccggagatccagtacacttccaactattacaagtctaataatgttgaatttgctgttaatactgaaggtgtatatagtgaaccccgccccattggcaccagatacctgactcgtaatctgtaa

SEQ ID NO: 43 - protein, 18 aa, synthetic construct
  source 1..18: note = T2A
EGRGSLLTCGDVEENPGP

SEQ ID NO: 44 - protein, 19 aa, synthetic construct
  source 1..19: note = P2A
ATNFSLLKQAGDVEENPGP

SEQ ID NO: 45 - protein, 20 aa, synthetic construct
  source 1..20: note = E2A
QCTNYALLKLAGDVESNPGP

SEQ ID NO: 46 - protein, 22 aa, synthetic construct
  source 1..22: note = F2A
VKQTLNFDLLKLAGDVESNPGP

SEQ ID NO: 47 - DNA, 54 bp, synthetic construct
  source 1..54: mol_type = other DNA; note = T2A
gagggcagaggcagtctgctgacatgcggtgacgtggaagagaatcccggccct

SEQ ID NO: 48 - DNA, 57 bp, synthetic construct
  source 1..57: mol_type = other DNA; note = P2A
gccaccaacttctccctgctgaagcaggccggcgacgtggaggagaaccccggcccc

SEQ ID NO: 49 - DNA, 60 bp, synthetic construct
  source 1..60: mol_type = other DNA; note = E2A
cagtgcaccaactacgccctgctgaagctggccggcgatgtggagagcaaccccgggccc

SEQ ID NO: 50 - DNA, 66 bp, synthetic construct
  source 1..66: mol_type = other DNA; note = F2A
gtgaaacagactttgaattttgaccttctcaagttggcgggagacgtggagtccaaccctggacct